European Patent Application EP 4 461 356 A2, published November 13, 2024. Title: METHODS OF TREATING AN ISCHEMIC DISEASE. Applicant: ELANI Dalia. The sequence listing filed with the application follows.

SEQUENCE LISTING (47 sequences)

SEQ ID NO: 1 - protein, 233 aa, Homo sapiens
MSTESMIRDVELAEEALPKKTGGPQGSRRCLFLSLFSFLIVAGATTLFCLLHFGVIGPQREEFPRDLSLISPLAQAVRSSSRTPSDKPVAHVVANPQAEGQLQWLNRRANALLANGVELRDNQLVVPSEGLYLIYSQVLFKGQGCPSTHVLLTHTISRIAVSYQTKVNLLSAIKSPCQRETPEGAEAKPWYEPIYLGGVFQLEKGDRLSAEINRPDYLDFAESGQVYFGIIAL

SEQ ID NO: 2 - DNA, 13361 bp, Homo sapiens
  source 1..13361: mol_type = genomic DNA
ctcctccagctcttcctgtcccgctgttgcaacactgcctcactcttcccctcccaccttctctcccctcctctctgctttaattttctcagaattctctggactgaggctccagttctggcctttggggttcaagatcactgggaccaggccgtgatctctatgcccgagtctcaaccctcaactgtcaccccaaggcacttgggacgtcctggacagaccgagtcccgggaagccccagcactgccgctgccacactgccctgagcccaaatgggggagtgagaggccatagctgtctggcatgggcctctccaccgtgcctgacctgctgctgccactggtgagaccagggacaaagggaagagtgggctggtgggcgaggcaccttccggctggcgtgggccctctccgggagggggccgagcctctcctgcccgggcctggtcctggcgccagcctcaggcctgcaggtcctaacctcagccactgccagtgtggggttccccattcatccgccttttggagtaggggctgcgctgaggcaggggaatgggagaagtttgaaagggagagagtaaaaggaagccctggcccctgacagcggtggaagtttgtgggcggccaagggaatgtgggcaggagataggcccagggtggggcagatttggcggggaaaagaagggagtgggagtaggaagattagtgctcggggagtccagacggttctgaattctgtccctccggtcagctggctggcctggagggtgttgggccgtggggaggcgaggctgcctgtggaacttggtggagcacaccctgtagggcaggattttggcggctggtgaagtgggggagtgagttgaggagtggggatgggctggtgtggtgggtttgggatgctcatggtgggaggtatttgagaatgggctgggacactggatggggcagggcaacccagtggacagtgtccccagtgccctggccaagccccggcctctcacctggggacattctttacccttttgcctgctgctaggcaggtagccgctgtgggactgagccttcccagggagctagtcctacccccacctggtcagtgtccctgggcctgtcctccagcttcccctccccgctgcttctcacagacctaaacaacaatcccttggtttcttattctacagttcagtttggggaagttggtagaaagttgttttcgtcactggaaaatgtccctttctctggcctcagccttgtttcaatgtatccttgatcgtcctccacgtcttggtccgggaatcatcctgttcagatgtcctgggcccatctagtcaggcagattttccctgccctgcccggcctctgaaggctgcgcctacctcccctctctttagtgccttatactcttcctctcctaccattcctttcttccagcaatctccccagactctcctcagacttctcagagcctctttttttgaaatcttttctcgctaatcctccttcccctcctctctgctccgctctggtcccggccccaggtccccaggcagcacgtctctggtcagggtctcactcttcttcttctgcctcctcctgcctccttagtcccacccgctcttcccttcttcccactgtccttcccccacggtctccccaccagccagctgccctgacatcctgcttctgttttctgtttgggggcggcccctggctccctcacatacctcctgcatgaacaagagcagcttatataacctaaccttccatgccttcgtttctttatctccaaaatgggtgtcacagtcttgacctcatactgttgttttgaagattgaatagactgatacatgttaagtgttcatttgatttattaagtgtgcgctctgggctagacactgtgataggtgctgggattacagcagagaacaaaatccctgcccacagctttgacagtccatcaggggaataggttgtagcaaatagaaagcactcaataaagtttttatattgctgtgactagtagtaattactgggtggctacctgtgttgggaaaacagagggtaaaggtagcctgaacaggtaaagggaagtgcctgcgtcctggggtgcttcagcccaggtgggattatgtctcctaagggacagaagcctggcctggagctggaggaaagggaaaacaaagggaatgcaacatccttctgaatttctcaccattcagtgggcaatgcagagctcacagtgtgtgtgtgtgtgtgtgtgtgtgtgtgtgtgtgagagagagagagagagagagagagaagtggggtaggggagtagggaagaatgatacaggagagactgtggcaaagcaaacaggattttgctgctctcaaagagcttacagcctagtaaccaagatggcttacagtgaaaaatgatttcagagcaatcccgaggaaaatatccacaaatgcattgtgatgtggtgtcctggagcaccagttgggaggaggaggaactggggaaggaggtgagccttagtccactgcctttccttgcttagcaggtctcagctcctgcgctcagctccagaaaattcaggagcttccccacgctgcttcagtgtccttcactgtgcaactgcagcactccctgtatagatctcagtgcctacaactgactgtctttgactcaagtgagagctcttgagagcacgagctgtgtattatccacctcagcatccctagcacccatacgggacctgtcacattaactgtgccccttaactatttgctgaaggaattaaggaacaagagatgtgtcagatgggatggcggagggaaagcctcatagaaaagtggatgtggagctgacatctgaagtcactgcctgtcagggtagctataaaggagggaagcagagttggatactgatgtgaggaagaggagaggaatggagagatgggattttgtgttgatgggcagggtggcaggaagccagacaccttggttcgggagtggaaaaaccatgttgagaaacactaagaaatgtgaatgggagaattagagggagtgggggagaggatggaggaagagtgttgaatatggttccaggtggaggaattcattcattcgtttattcagaagctgttctcctagggcacattctgtgcccagactgtgattagaagtgaggtgaggcatctcagatgggtgctgtggttcatgcctgtaattccagcacttcaggaggccgaggtgtgtggattgcttgagtccaggagttcgagaccagcctgggcaacacagcaaaaccctgtctctacaaaaaatacaaagattagcggggcatggtggggcgtgcttgtcatcccagctattcgggagactgagctcgggaggacggcttgggcccaggaggtggaggttgtagtgagccctgaccacaccactacattccgtcctggtggtgaaggttgcagtgagctatgattgtgccactgcacttcaccctgggtgacagagtgagaccctgtttcaaaaaaaaaaaaaaaaaagtagtgaggcatctgtggaagtcttcagatcatttccatgaccatggaaatgctgtttggagccaggccctggagatggagaggaaggttcacacacttgtgcgtgcaagttaaagcctgaatgaagatttaaaaagtgtgtaggacggatgggagcaggagagaggctagaagacacttgcaataacccaggtgtgaggcaacccaggaatgcggagaggaccgagagatcacagggggaggcctcgcaagatgaactgacacatgggatggcggcagggatagggatggggccctggggagagagcgtggcaagttctcagcattcgtccgggaagtcgatggtgtgtcatttgtctaggtgaggagatggatgaattccgtctggggcatgttaagggtcagggaaatggtcatgtggaagggtgcgcctaccaagctggaggagaggtgctgcaacttctttctgcctttgtatcattcagacacactgtgttcactcatcagtggttctcaaaaggagaggagcacaccagactcttaagtaagggtgtgtgtgcttgtgtgtggggaggtggggggatggtctgaaaactctcccccggagataaatatattcctaccaggggtgctgtctcctcacctccctctttgggaatcactggcttctactagagtggaagacagatgtatcattagatcgatcagttgatccatatttatctgctcccagtctggaggtctggttctgggagctgagaggacaccaggggaggataagacactttctgaccaagacattttttgatctctcatcttataaggttcgtggtcactttggggagatcatatctgtcacccaacataaccatattatgataagagccaaaagtagatagggtcagttcacgtgcttcgagttcacagggactatgggtctaaggagccggggtggaggaaacagacatcgtcaatggtggcttcacgggagggagatgggatctcaactgggcccttggaggagaagctgccacgacctcccccaacaccttgacattaaatgaacagacacatgaatgagggggaaaggaagactaattgggtccctgcaaggtggctggatcggggtcagaccacaaggccgatctcagcgtcgcctccccactctgcagccccagcacaggaagtcacactttaaagcctcctctggcggaaattgtgggggagttggaggggtgttgggccaccccctcaactgtctctccacaggcaccccagcttcctgcccttctgctccaggctggagtctgggcctaaagagctcacctcctgtttctcctgttttgcttcatttacgcaactgctgaggactgggcttactggggccagctggtgccagcagtggtgcccagtggtggggagtctgagggccctggctcctagggatcagagagggctgacctggagcattctgggggccaggggaagcctaggaagcagggctggttcttccatccggcatcccttcttgcctgctccctcgttcctggaagtgggtgttcagggctctggaggctttcctgtattgccagtgggcttggggagggtctgtggagactcagaactggccttgtttcctaaggattgtctggggaccccagggaggcccccaaacccagcacaactggtcagaaccagccaggctgtgggaatgcggtgaacccagggtgggagggcagccttggcttgcttcctgctgggactggggagtgttgggggatggagtgagagctcacggaatgggtttagctgttggagacttgttgaactgggaggaggagctggggcggggcctcagctaaaggccgctgaggggctaggaggagccaagtggccctcagggaagggagggcacagacctgatgggcggaagccagggtcgagggagacttcccttcgggatggaatggggagagggaggcatttcccggaacatgtgggccaagtgggacaagggtctgtggcctggctctttgcatggggaggggatggatgggggttgagtggggatgggaaggagggacttggccataggaagaagggattagatggagtcccacttgcatgcaggctggtgccttctgcctttctgctgactcatgacccttgaggagctggggaagctgctagttccctctcccctccctaggtctccctccctctggcctgagtcactggggcggagttgctgggaaaagatttccctttcccggatctgacttaacccccagagtgctggaaagagaagggaacacgtggcctgagaaagcctctctccctccctccctccagggaggctcatcccccactggccagaggtccctgaaaagctccctttaaggctgtctggggctggcgtcccccagttcttcatcatgactctgcctcaagccccctggatgggattcaaagtaccagtgaccttaggtgctccagtggcttcttcggggaaaggaaccacactttcaggactgggaagttcttcccatcaccaccccaaacccttcctgttgccctggaagccccagtcctgttctcagcagaggtggcacggtgttggctggtgcgggcaggggaaggttgttgtcctctgagcaggggcacacgcctccacctgcgggggctgctgttgtgtttctgtgtgtggcttcccctgtttgcggctgaggcttgaacttccgggcctgcacagcttacagctgcagcgtctccccgtggctgactcagggtgactggcctcctgctccgaaatgtggagttggtgaggctgggtggctgtgggctgcctgaccctccttccctgccctagggtttctgtgatctggtgagtcagttgctccccagtgtttaacagacattgaggacaccctcttatctttacacaaagtgtctcttatagtagaaaaaaaaaatgaagcccagggaaaaccagaaatgaagctggcagagatcaaagtccaagttagagctaaatattcactcctggctttgctttcctggcactgatgccggaacaggacaagccatttagctgctgtggggttggcctgagactgcaaagcacaccttccagaatgccatggtgtgcagggggctccaggactccccagcacgccctcagctctgacctgacagtcatccaagctgggtcgctagccttggccagctctatttgcctatgtcctgcacacctttgcccactcctgcccccgtctcaactttgtcccccgtctacccatgcaggatccccaacctttcccttttactctcctccccatttgtccttgccaaccccgggtgtttgtaaattttgaggtggaggggatgggccagggaatgtgagggcggaggcagattgaggtttgatacaaacatgtaaataaacttccttcttctgtccactccccaggagtggtgctcacgggaacatcactcgcccccaccgccagctgactttttcagaaagcttttcatggtgtaacatattcctgggatgtgcatagatcctcattgtttacctctgtgaatgttcgcaaagcgatcacacggtgaacccagcacccagatggagaaacaccgccccaatctttagggctgcttgttggaagaaggggccatcactgaagtaacctgccaattcccaatcaaaaacacatcctttcaacatctgccctgtgtccagcactgttagctgctgtgggggatttcacagtaaggataaaatacagggctgggctcacgcctgtaatcctagcactttgggaagccaaggtgggaggatcacttgagcccaggattttgagaccagtctgagcaacgtaacaagaccctgcctctactaaaaataaaaaaaaattagctgggcatggtggttcacggccgtagtcccagctattcaggaggctaaggtgggaggactgcttgagcgtgggtggtggagggtgcagtgattgcatcactgcactccagcctggacaacagagcaagatcctgcctaaaaaaaaaaaaatacagcttagatctggggcctactagctttgagttgagggaacaaaaatgaacacacaggacaactagagaacaattaagcatcagattgtatggccccaactgtctaagtttcaaggaagaactctaaacttagtgagtggcgtggcctgggcggaatgtttcactgaggaaggacttgagccagggaagttttagatctgctacccctaagcttcccatccctccctctcttgatggtgtctcctctatctgattcttccccaggtgctcctggagctgttggtgggaatatacccctcaggggttattggactggtccctcacctaggggacagggagaagagagatagtgtgtgtccccaaggaaaatatatccaccctcaaaataattcgatttgctgtaccaagtgccacaaaggtaggggcaagtggaaacggtgaatgccctcaggtctggggtgctgcttctttctctgcttcttccagttgttcttccctaactttgctgtctctcctgggctgggattttctccctccctcctctcctagagacttcagggaatcggccctggctgttgtccctagcatggggctccttccttgtgttctcacccgcagcctaactctgcggccccattcacaggaacctacttgtacaatgactgtccaggcccggggcaggatacggactgcagggagtgtgagagcggctccttcaccgcttcagaaaaccacctcagacactgcctcagctgctccaaatgccgaaagggtgagtgtgcacaggcaggagagtcaggcgggtcttgagtggtgtgtgggtgcctgtctatgtgcaggctggtgggtgtgggcaggaaggtgtgtgttttggtgggacactgcatggatgtgagtgtgtattacagagacacacacttaggggtatgtcaggaaggggatgcagggacaggaggatgcaggactcataccccatcttctcccctcaccagaaatgggtcaggtggagatctcttcttgcacagtggaccgggacaccgtgtgtggctgcaggaagaaccagtaccggcattattggagtgaaaaccttttccagtgcttcaattgcagcctctgcctcaatgggaccgtgcacctctcctgtgagcgcagctctcctgaggccaagccctctccccaccccaggggttggccccttccccatgcggtggcacttcctttccttccccctcctgtattctgtgggtctgacaaccaactcctctctggccgcccccaccctgtccctcgtcacttcctctgtcctgtggggtgggggtgcaggcgcttctcctttagctgtgccgcacttctccctacaggccaggagaaacagaacaccgtgtgcacctgccatgcaggtttctttctaagagaaaacgagtgtgtctcctgtagtaagtgagtatctctgagagctgctgggcactggatggtggcatgggttgggacgggtgactggtgggaaccattagctgggcaacagatgccaggatgccccagagtgctcagggtcctactggctgagtaggagacacttcgttaagacaccaggcagtccttccccttgctcttcaaatctgaagaagtctttgaggatggaagatcatgccccaagggctggcagcccttccaactcagatatgtagattcttggatctacgatagctcattggttctaggacatacactcttatagctctgaaatcaaacctcctataactggtgactcatcatggttgaattggcagctctgtttgcgtctgggtagtaatgtaaagaaaagtgccttttattcttgatggcgtcttaggtttgatgcaatatggtatttcctcattagtcactgtccaggcctccttactcctggctccacagaggctgttcttgtcactcacttgcaaagaataaactctgagggctctcagagtttgaaccccagcatagccacttactggctatgtgacgttgggcaagtttcttaacatctctgagcctgacttttcttttggtgttttttttttttttttttttttgagacagggtttcactctgtcacccaggctggagtgcagtggtgcaaccgtggctcagcctccacctccagggctcaagccatcctcttgccttagcctcctgagtagctgggattagaggcacacaccactacacccagctaatgttttactttttgtagagacagggtcctactatattgcccaggctggcctcggactcctgggctcaagcgatcttccgcctcagcctcccaaagtgctaggattacgggcatgagccaccacgcctggcctgggccttagatttcttatatttaaagtaagcataatgacattcatttggtgaatttgtgagaaccaaaaacaaagaaacaaacaaaacctacaacacgtctgacacaaaactatttattttccattaatcttcttttttttttttttttttttttttgacacagagtcctgctctgtcgcccaggctggaatgcagtggcgcgatctcggctcactgcaacctctgcctcccagattcaagcaattctcctgcttcagcctcccaagtagctgggattacaggcacgtgccaccatgcctggctaatttttgtatttttagtagagatggggtttcaccatcttggtcaggctggtctcaaactcctggtgatccacctgcctctgcctcccaaagtgctgggattacagccgtgagccactgcacccagccggcttcatctcttcttgaaatcacttttataccattctatgtggttctcaccatgagcttgagtggtgggctaaagtgcctctccctgctttcagcttcctgctgggaactcactctctcaagttccttccagcaccaccccatagagttcccatcactccacactgtccagtgacaactcccaacatggaagatctgctagttctacagggtgctctctggctgccccagtaacatgtgtttttaaatttttcacatgcatgtttgaccccgactccccgaagtcaggtactgtaactagcagtgtcatttaagaaaaagccctttaacctctctttgccaaaggattcttatcagcaaaacagtgatgaaacaacaatcccataacagctagctggctaccttctcaagcacttattaaatgaggcataatgattttgcttaatcctcaatcctgagaggtgggcgatccctgtggtgatgaggaaaccgaggcttgggggttaatggcttgcctagattcacactgctagccaaggaatgaactggaatttacaccctgaccctgactgcttttcacattttctacacagccttttcaagatccctgccaattctaaaattaaatgattctatgattaactgtgtttcattcttctgcatcagttcccaaaacaaattatatcaagagacagcaaaaatatttgtaaagaaaggatgtccaacaatctgtgtggttgtttttctgtgttcctccaatggtagggcctctgttcaccagtgccgtctcttcttttagctgtaagaaaagcctggagtgcacgaagttgtgcctaccccagattgagaatgttaagggcactgaggactcaggtgaggagaagtgacctggtgcccatgctcacctgccctctccctcttcttgcccccacccgtccatccatcccacccatccatctatccctgcggcccccctctgcccgctcctctgaccaacacctgctttgtctgcaggcaccacagtgctgttgcccctggtcattttctttggtctttgccttttatccctcctcttcattggtttaatgtatcgctaccaacggtggaagtccaagctctactccattggtgagtgggggctttgggagggagagggagctggtgggggtgagggaggacatgggtgggtgcgatggacatgtgtggagggaggtgaggagtgtcccctcagttcataccgctggggactctgggcagaaggtggccctggatggctggggagatgtcgagctgcatcagtagctctctcgtccctggggccacataggccctgaggcatgtcaccacaagtccccactgccagctgagtccagggtgccagggctgagagaggaagtgaaatttatgatgctttctttctttttcctcagtttgtgggaaatcgacacctgaaaaagaggtgagatgaaatgagagagttactcccaaatgtccctgaccattccttataattgcctaatgctcagatcccctggaatcatccttcactttccgggggctcgcctcattccctctaagtcccaacccccacgtagaataaagagggccggggctggttttcgctgccgcactaatgttgcgccaccttctctctttcagggggagcttgaaggaactactactaagcccctggccccaaacccaagcttcagtcccactccaggcttcacccccaccctgggcttcagtcccgtgcccagttccaccttcacctccagctccacctatacccccggtgactgtcccaactttgcggctccccgcagagaggtggcaccaccctatcagggggctgaccccatccttgcgacagccctcgcctccgaccccatccccaacccccttcagaagtgggaggacagcgcccacaagccacagagcctagacagtgagtttctcccgcggctggagacgaggaggctgggggagggccgggggagcgcgggaggcgctcccagaggggaccacgagaggcggagggcgcgggatgcggggcggggcctggggttgccgcccgaggctcaccggcccgcgtccccgcagctgatgaccccgcgacgctgtacgccgtggtggagaacgtgcccccgttgcgctggaaggaattcgtgcggcgcctagggctgagcgaccacgagatcgatcggctggagctgcagaacgggcgctgcctgcgcgaggcgcaatacagcatgctggcgacctggaggcggcgcacgccgcggcgcgaggccacgctggagctgctgggacgcgtgctccgcgacatggacctgctgggctgcctggaggacatcgaggaggcgctttgcggccccgccgccctcccgcccgcgcccagtcttctcagatgaggctgcgcccctgcgggcagctctaaggaccgtcctgcgagatcgccttccaaccccacttttttctggaaaggaggggtcctgcaggggcaagcaggagctagcagccgcctacttggtgctaacccctcgatgtacatagcttttctcagctgcctgcgcgccgccgacagtcagcgctgtgcgcgcggagagaggtgcgccgtgggctcaagagcctgagtgggtggtttgcgaggatgagggacgctatgcctcatgcccgttttgggtgtcctcaccagcaaggctgctcgggggcccctggttcgtccctgagcctttttcacagtgcataagcagttttttttgtttttgttttgttttgttttgtttttaaatcaatcatgttacactaatagaaacttggcactcctgtgccctctgcctggacaagcacatagcaagctgaactgtcctaaggcaggggcgagcacggaacaatggggccttcagctggagctgtggacttttgtacatacactaaaattctgaagttaaagctctgctcttgga

SEQ ID NO: 3 - DNA, 2258 bp, Homo sapiens
  source 1..2258: mol_type = genomic DNA
ctcctccagctcttcctgtcccgctgttgcaacactgcctcactcttcccctcccaccttctctcccctcctctctgctttaattttctcagaattctctggactgaggctccagttctggcctttggggttcaagatcactgggaccaggccgtgatctctatgcccgagtctcaaccctcaactgtcaccccaaggcacttgggacgtcctggacagaccgagtcccgggaagccccagcactgccgctgccacactgccctgagcccaaatgggggagtgagaggccatagctgtctggcatgggcctctccaccgtgcctgacctgctgctgccactggtgctcctggagctgttggtgggaatatacccctcaggggttattggactggtccctcacctaggggacagggagaagagagatagtgtgtgtccccaaggaaaatatatccaccctcaaaataattcgatttgctgtaccaagtgccacaaaggaacctacttgtacaatgactgtccaggcccggggcaggatacggactgcagggagtgtgagagcggctccttcaccgcttcagaaaaccacctcagacactgcctcagctgctccaaatgccgaaaggaaatgggtcaggtggagatctcttcttgcacagtggaccgggacaccgtgtgtggctgcaggaagaaccagtaccggcattattggagtgaaaaccttttccagtgcttcaattgcagcctctgcctcaatgggaccgtgcacctctcctgccaggagaaacagaacaccgtgtgcacctgccatgcaggtttctttctaagagaaaacgagtgtgtctcctgtagtaactgtaagaaaagcctggagtgcacgaagttgtgcctaccccagattgagaatgttaagggcactgaggactcaggcaccacagtgctgttgcccctggtcattttctttggtctttgccttttatccctcctcttcattggtttaatgtatcgctaccaacggtggaagtccaagctctactccattgtttgtgggaaatcgacacctgaaaaagagggggagcttgaaggaactactactaagcccctggccccaaacccaagcttcagtcccactccaggcttcacccccaccctgggcttcagtcccgtgcccagttccaccttcacctccagctccacctatacccccggtgactgtcccaactttgcggctccccgcagagaggtggcaccaccctatcagggggctgaccccatccttgcgacagccctcgcctccgaccccatccccaacccccttcagaagtgggaggacagcgcccacaagccacagagcctagacactgatgaccccgcgacgctgtacgccgtggtggagaacgtgcccccgttgcgctggaaggaattcgtgcggcgcctagggctgagcgaccacgagatcgatcggctggagctgcagaacgggcgctgcctgcgcgaggcgcaatacagcatgctggcgacctggaggcggcgcacgccgcggcgcgaggccacgctggagctgctgggacgcgtgctccgcgacatggacctgctgggctgcctggaggacatcgaggaggcgctttgcggccccgccgccctcccgcccgcgcccagtcttctcagatgaggctgcgcccctgcgggcagctctaaggaccgtcctgcgagatcgccttccaaccccacttttttctggaaaggaggggtcctgcaggggcaagcaggagctagcagccgcctacttggtgctaacccctcgatgtacatagcttttctcagctgcctgcgcgccgccgacagtcagcgctgtgcgcgcggagagaggtgcgccgtgggctcaagagcctgagtgggtggtttgcgaggatgagggacgctatgcctcatgcccgttttgggtgtcctcaccagcaaggctgctcgggggcccctggttcgtccctgagcctttttcacagtgcataagcagttttttttgtttttgttttgttttgttttgtttttaaatcaatcatgttacactaatagaaacttggcactcctgtgccctctgcctggacaagcacatagcaagctgaactgtcctaaggcaggggcgagcacggaacaatggggccttcagctggagctgtggacttttgtacatacactaaaattctgaagttaaagctctgctcttggaaaaaaaaaaaaaaaaaaaaaaaaaaaaaaaaa

SEQ ID NO: 4 - DNA, 2102 bp, Homo sapiens
  source 1..2102: mol_type = genomic DNA
ctcctccagctcttcctgtcccgctgttgcaacactgcctcactcttcccctcccaccttctctcccctcctctctgctttaattttctcagaattctctggactgaggctccagttctggcctttggggttcaagatcactgggaccaggccgtgatctctatgcccgagtctcaaccctcaactgtcaccccaaggcacttgggacgtcctggacagaccgagtcccgggaagccccagcactgccgctgccacactgccctgagcccaaatgggggagtgagaggccatagctgtctggcatgggcctctccaccgtgcctgacctgctgctgccactggaacctacttgtacaatgactgtccaggcccggggcaggatacggactgcagggagtgtgagagcggctccttcaccgcttcagaaaaccacctcagacactgcctcagctgctccaaatgccgaaaggaaatgggtcaggtggagatctcttcttgcacagtggaccgggacaccgtgtgtggctgcaggaagaaccagtaccggcattattggagtgaaaaccttttccagtgcttcaattgcagcctctgcctcaatgggaccgtgcacctctcctgccaggagaaacagaacaccgtgtgcacctgccatgcaggtttctttctaagagaaaacgagtgtgtctcctgtagtaactgtaagaaaagcctggagtgcacgaagttgtgcctaccccagattgagaatgttaagggcactgaggactcaggcaccacagtgctgttgcccctggtcattttctttggtctttgccttttatccctcctcttcattggtttaatgtatcgctaccaacggtggaagtccaagctctactccattgtttgtgggaaatcgacacctgaaaaagagggggagcttgaaggaactactactaagcccctggccccaaacccaagcttcagtcccactccaggcttcacccccaccctgggcttcagtcccgtgcccagttccaccttcacctccagctccacctatacccccggtgactgtcccaactttgcggctccccgcagagaggtggcaccaccctatcagggggctgaccccatccttgcgacagccctcgcctccgaccccatccccaacccccttcagaagtgggaggacagcgcccacaagccacagagcctagacactgatgaccccgcgacgctgtacgccgtggtggagaacgtgcccccgttgcgctggaaggaattcgtgcggcgcctagggctgagcgaccacgagatcgatcggctggagctgcagaacgggcgctgcctgcgcgaggcgcaatacagcatgctggcgacctggaggcggcgcacgccgcggcgcgaggccacgctggagctgctgggacgcgtgctccgcgacatggacctgctgggctgcctggaggacatcgaggaggcgctttgcggccccgccgccctcccgcccgcgcccagtcttctcagatgaggctgcgcccctgcgggcagctctaaggaccgtcctgcgagatcgccttccaaccccacttttttctggaaaggaggggtcctgcaggggcaagcaggagctagcagccgcctacttggtgctaacccctcgatgtacatagcttttctcagctgcctgcgcgccgccgacagtcagcgctgtgcgcgcggagagaggtgcgccgtgggctcaagagcctgagtgggtggtttgcgaggatgagggacgctatgcctcatgcccgttttgggtgtcctcaccagcaaggctgctcgggggcccctggttcgtccctgagcctttttcacagtgcataagcagttttttttgtttttgttttgttttgttttgtttttaaatcaatcatgttacactaatagaaacttggcactcctgtgccctctgcctggacaagcacatagcaagctgaactgtcctaaggcaggggcgagcacggaacaatggggccttcagctggagctgtggacttttgtacatacactaaaattctgaagttaaagctctgctcttggaaaaaaaaaaaaaaaaaaaaaaaaaaaaaaa

SEQ ID NO: 5 - DNA, 2374 bp, Homo sapiens
  source 1..2374: mol_type = genomic DNA
ctcctccagctcttcctgtcccgctgttgcaacactgcctcactcttcccctcccaccttctctcccctcctctctgctttaattttctcagaattctctggactgaggctccagttctggcctttggggttcaagatcactgggaccaggccgtgatctctatgcccgagtctcaaccctcaactgtcaccccaaggcacttgggacgtcctggacagaccgagtcccgggaagccccagcactgccgctgccacactgccctgagcccaaatgggggagtgagaggccatagctgtctggcatgggcctctccaccgtgcctgacctgctgctgccactggtgctcctggagctgttggtgggaatatacccctcaggggttattggactggtccctcacctaggggacagggagaagagagatagtgtgtgtccccaaggaaaatatatccaccctcaaaataattcgatttgctgtaccaagtgccacaaaggaacctacttgtacaatgactgtccaggcccggggcaggatacggactgcagggagtgtgagagcggctccttcaccgcttcagaaaaccacctcagacactgcctcagctgctccaaatgccgaaaggaaatgggtcaggtggagatctcttcttgcacagtggaccgggacaccgtgtgtggctgcaggaagaaccagtaccggcattattggagtgaaaaccttttccagtgcttcaattgcagcctctgcctcaatgggaccgtgcacctctcctgccaggagaaacagaacaccgtgtgcacctgccatgcaggtttctttctaagagaaaacgagtgtgtctcctgtagtaaagtcctgctctgtcgcccaggctggaatgcagtggcgcgatctcggctcactgcaacctctgcctcccagattcaagcaattctcctgcttcagcctcccaagtagctgggattacagctgtaagaaaagcctggagtgcacgaagttgtgcctaccccagattgagaatgttaagggcactgaggactcaggcaccacagtgctgttgcccctggtcattttctttggtctttgccttttatccctcctcttcattggtttaatgtatcgctaccaacggtggaagtccaagctctactccattgtttgtgggaaatcgacacctgaaaaagagggggagcttgaaggaactactactaagcccctggccccaaacccaagcttcagtcccactccaggcttcacccccaccctgggcttcagtcccgtgcccagttccaccttcacctccagctccacctatacccccggtgactgtcccaactttgcggctccccgcagagaggtggcaccaccctatcagggggctgaccccatccttgcgacagccctcgcctccgaccccatccccaacccccttcagaagtgggaggacagcgcccacaagccacagagcctagacactgatgaccccgcgacgctgtacgccgtggtggagaacgtgcccccgttgcgctggaaggaattcgtgcggcgcctagggctgagcgaccacgagatcgatcggctggagctgcagaacgggcgctgcctgcgcgaggcgcaatacagcatgctggcgacctggaggcggcgcacgccgcggcgcgaggccacgctggagctgctgggacgcgtgctccgcgacatggacctgctgggctgcctggaggacatcgaggaggcgctttgcggccccgccgccctcccgcccgcgcccagtcttctcagatgaggctgcgcccctgcgggcagctctaaggaccgtcctgcgagatcgccttccaaccccacttttttctggaaaggaggggtcctgcaggggcaagcaggagctagcagccgcctacttggtgctaacccctcgatgtacatagcttttctcagctgcctgcgcgccgccgacagtcagcgctgtgcgcgcggagagaggtgcgccgtgggctcaagagcctgagtgggtggtttgcgaggatgagggacgctatgcctcatgcccgttttgggtgtcctcaccagcaaggctgctcgggggcccctggttcgtccctgagcctttttcacagtgcataagcagttttttttgtttttgttttgttttgttttgtttttaaatcaatcatgttacactaatagaaacttggcactcctgtgccctctgcctggacaagcacatagcaagctgaactgtcctaaggcaggggcgagcacggaacaatggggccttcagctggagctgtggacttttgtacatacactaaaattctgaagttaaagctctgctcttggaaaaaaaaaaaaaaaaaaaaaaaaaaaaaaa

SEQ ID NO: 6 - protein, 455 aa, Homo sapiens
MGLSTVPDLLLPLVLLELLVGIYPSGVIGLVPHLGDREKRDSVCPQGKYIHPQNNSICCTKCHKGTYLYNDCPGPGQDTDCRECESGSFTASENHLRHCLSCSKCRKEMGQVEISSCTVDRDTVCGCRKNQYRHYWSENLFQCFNCSLCLNGTVHLSCQEKQNTVCTCHAGFFLRENECVSCSNCKKSLECTKLCLPQIENVKGTEDSGTTVLLPLVIFFGLCLLSLLFIGLMYRYQRWKSKLYSIVCGKSTPEKEGELEGTTTKPLAPNPSFSPTPGFTPTLGFSPVPSSTFTSSSTYTPGDCPNFAAPRREVAPPYQGADPILATALASDPIPNPLQKWEDSAHKPQSLDTDDPATLYAVVENVPPLRWKEFVRRLGLSDHEIDRLELQNGRCLREAQYSMLATWRRRTPRREATLELLGRVLRDMDLLGCLEDIEEALCGPAALPPAPSLLR

SEQ ID NO: 7 - protein, 347 aa, Homo sapiens
MGQVEISSCTVDRDTVCGCRKNQYRHYWSENLFQCFNCSLCLNGTVHLSCQEKQNTVCTCHAGFFLRENECVSCSNCKKSLECTKLCLPQIENVKGTEDSGTTVLLPLVIFFGLCLLSLLFIGLMYRYQRWKSKLYSIVCGKSTPEKEGELEGTTTKPLAPNPSFSPTPGFTPTLGFSPVPSSTFTSSSTYTPGDCPNFAAPRREVAPPYQGADPILATALASDPIPNPLQKWEDSAHKPQSLDTDDPATLYAVVENVPPLRWKEFVRRLGLSDHEIDRLELQNGRCLREAQYSMLATWRRRTPRREATLELLGRVLRDMDLLGCLEDIEEALCGPAALPPAPSLLR

SEQ ID NO: 8 - protein, 302 aa, Homo sapiens
MQWRDLGSLQPLPPRFKQFSCFSLPSSWDYSCKKSLECTKLCLPQIENVKGTEDSGTTVLLPLVIFFGLCLLSLLFIGLMYRYQRWKSKLYSIVCGKSTPEKEGELEGTTTKPLAPNPSFSPTPGFTPTLGFSPVPSSTFTSSSTYTPGDCPNFAAPRREVAPPYQGADPILATALASDPIPNPLQKWEDSAHKPQSLDTDDPATLYAVVENVPPLRWKEFVRRLGLSDHEIDRLELQNGRCLREAQYSMLATWRRRTPRREATLELLGRVLRDMDLLGCLEDIEEALCGPAALPPAPSLLR

SEQ ID NO: 9 - DNA, 12761 bp, Mus musculus
  source 1..12761: mol_type = genomic DNA
cgctcttgcaacaccacccccgccactctcccttcccctcctaccttctctctcccctcagcttaaattttctccgagttttccgaactctggctcatgatcgggcctactgggtgcgaggtcctggaggaccgtaccctgatctctatctgcctctgactttcagcttctcgaactcgaggcccaggctgccatcgcccgggccacctggtccgatcatcttacttcattcacgagcgttgtcaattgctgccctgtccccagccccaatgggggagtgagaggccactgccggccggacatgggtctccccaccgtgcctggcctgctgctgtcactggtgagatgggagactggaggggagggtgggttgctagcgaggcgccgggcaggagtgggcttgtactaggggtagagatgggggcaggggcttctgtgctttagtttgacgccaggtttgctgtgcctcacctggggctgccctgagatgtggaagggagaaatctgagagggagagaatctggcaagccaagctggcaagcctgggcccctgacagtcaaggtcctggcccgtgttgggctgtggtcaggccagctgctcggccagtggagttagacggagaagccttctttctctggccgaggttgaacagcgtggggcagggtgttggaagactgggtgctaggagaaccgctttggcgggacgagtttgggaaagcgtgcttgggagtggacccgaaactggacaaagctgggcagccttccggtcccagacttctccctgagacagcctctgaccttctgccgcctccatttctgcttccagacaagaggtccctcctggcgtgaccctccttaagtagctaatacctctttatctaggccatgtatcctcctgctccctccccacagacccaaaagtcagtctcacggtttccaattccacagttccaattggggaagttggtagcagcttgttttcgtcactggaaaatgtacttttctctggcctcggcctagtgttcatgttctcttgatttctgtgtgtccataattattctgtgtagatcctgggggctccctggctgtctgggtgggctgtaccatcggcgcagtgttctctgggtcctgcctctccctggcccagcgttatccctgagacctgcctttttctccctcccctttcactcctcattctcttctggtcagtctccagagcctccttgcgggggtggggtgggggggtgggggtggctcctttgtgtctattcccttccctttctctacacaccattctaaagcagtggtcctagaaccctgcctgggtgtcacctcccttctcctggtcctgtcctgtctcccagtctctcctgggagacttgtcaaggctgcccctctggctgttctccaactcccccacccacttaattcttttctctttaggggtagatcacctggatttagggctcagcccagcacccttaccctcatgaacgcaggcatgtgatgtgactcccccgctttttgtttcttttatttccaaaatgtctacaatgatcagtacctcatagttgttattaagattgagtagatggatttgtgttaaatatttattcatttccttccctgctaggtccaattcagattaggtgaatgatcccaaaggggagtaagaagtatgccacaaacagaaaggactcagcttggcttctctcttctcatctctagcagtgatactcgtcactactcacgtcactactcattgtgacggtagatgtcacaataactgtcagagtgcagtggcccagctaggtagaggagagaggctgagccagttgtggaggcccaggtgagggtgggggcaccgtgaacagaagcagatcctgaagacaaggcacacggaaggctactgaagtctacatggggctggccactgccttatcagtacagagcacagtgcctgtgaggtgttcaggtaggacgaggtgctgaggtcatgaggcagtgatggccgtggcagggatgtggcaaggccaagaagactttgctatttttaaaaagtttcagtacaggagtggaaatgactttagaatactctggaggaaaagacgttccaaggccttggtgatgtactatcccagaggcagaactgggggaggagggtgggctatatgccaactgtcttcttgcttaatggcctttgcctgtctgctgggctgagcttgcctgcatagaccctaaggctcatagtgtgttatcatctttggctcatggagagctcttgaaactgtgagctatgtcccatccccagcacctatccaggccctgaaaaagaaaccttgaccgttgactaatggcttaatcaattcaggaacaagagattggtcagatgggaacaaggcgggtgttgcatagaaaggaggacttggaactggtgtgcagaagccaggaggaggaagaacagaggagttgggcgcctgggttgggggaatggagaggtgggactttgaagtcacagaagctgaacatctcagctcggggtggagtggccatgttgagaaatgtgacagagagagaagggcactctggcgtttgtgaaaaagaaccttgagccagtcaccttggggcatgcctgttatcctggaacttgggagatggaggccagtgctcagatcgaggcccagttttggctatatagggagctggaggccagcctggatgactgagactgtgtcttaaaaacaccaaaaagaaataaagagtcatgcttaaggacctaggtgggggcctgttttcctctttccctccctctctccctcccttcctccctccctccctccctcctccctccccttcctcctttgctatccaccaagcagtctggccagactgtgttccaaagaacagtgagtttctcagatgtatgtgctcatggaaggatttatccatggaaatgatgtttgaagccaggccctggaggtgcagaggaagattcacacccaggtggtacaagttgaagcctgaatgtagataagaaactatgtaggtagcctcagcccctgcaaaggtttgaggcaggcacatcacttgaaccagaaggttcgtggcagcctgagccacatagtgaagccctgagacaccactgtggagtaggaaggagaaaggcagttgtaaaaaccagggctccgggtgtggggtaaagggtggagaggttccagaaggactgactgatgagtcttagggctgttgcagagtttgcagcattggtaccaagaagtcggtggtgtgacatctaggcaaggagcttggtgagctcagctgggggcaggttaaagtaggtcactggctggctaagtggaagtgtggttgtgctgtctggagcagcccttctcagcctttcttccagctaattccagctgcatggctcgtcagctggactctgcaggagatgagcaaatgtggcagaattgtcaccagggacatgtgcacgagtgtgcccgtgtgtggggaaggggatgcacagcttctaaaatacctcccagaggcagagtgtgtttgaggcagggggatgctgcttccttccatccggctccctgactggaaggcacctcagtccctcaggtctgcaggcctggctctgggtgatgtgaccaagacatgctctgatctcttaactcagagggtttgtggtctgtctggggagattgtatctactcatttgaaataactatagcttctgataagagcccagagtagatatggatagttcgtgttattcaaccagaacaggcggctaggtatccgaggagcttgggtggggagacatgaatcatcgacggggggcttcgtgggtggaaggtaggattgcggcagcgtggcagcgctctctgaggaggtcacaccgaagagctcctcaccaccgtaggtcttgacattaagtggaacacagtttaacctaatgtgcacgctgatgtggggcttagtgagtgggtccccaaaaggtggctgggtcaagtttgaccacagggtccatttcatcttcgctcccctactcagcagccccggcacaggaagtcacactttaaggcctctctaggcggaagctgaggagtagttagagaggccttgccacctcctcagccatctctcctctcctcaggcaccccccagcatcctgcccctcctctgctccaggcattcaagtttgggccaggacctgtgtcccttgtcccttgttggcctcacaatgcaactggtaatagggtgcctattgaaagagccagagggccctggaatccctggagcatgtgagatgagagagctggctctgcacctgctccttctcttttgttaccttgtttttgttgagagtagacctggctgtcctagaactcacattgtagagcaggctggccttgaacccagggatctgcctgcctccacctctcagagtgcctggattaatgtctagcttcctccatctcttctaaccttaagagggctgtgatttttgttccatagctacttgacctggggagaactggccctgtctcttaaaggttgtctagggagcatccaaacccaatgcaagtggccagaaccaggcaggctatgggaatgtggtgaactagggcgggagggcaccctggatttgattcttgttgggattggggagtgtcaggggctgccaaaggcccagggagccagggagcagggatcctgggaaaggctttatcagctgaagacgatgttgtttccctttgaggagggatcaaggcagctccaagtccaaaggaaggatgtcagagatggaggaggtagatcctctgggaggagcttactggcctgacagggaagccaggggtcagaaagacttccctttgggatgggatggaagagggaggcattttcccgaaatctgagcccagtgggacaggggttcattgcctggacgaatggtctgagtgggggtgggtgagagagagagagagactgtgcacccaggagggagcagatggggttccacttgctgctggttggcttttctgctgattcacagcccttgttgagccgggaagctgcagttccctgtccactgtcctagatctccctccctggcctgagtcactggggcggagctgctgggaaaagatttccctttcccggatttgacttaacccccagagttctgcaaaggaaggacacgtgaccaaagaaacaggctccttctctggaggctcgtccatcgctggttgagactcgcccccacccccacccccgcaaggccgttcttggcctggagcccacatctacctcttcctgacactgcctgatctgttggtttggcttcaggttctctgatggggttggaagtaccactgaccttaggtgctccaagcatttcttcttcggggaaaggaaccacactttcatgattgggaagttcttatcataactaacccttcctgtcaccctggaagcctctgtgtgtcgtgaggggtgggggtgcacccctgcctgagagattgctggtgtgctttctgtgtgtggcttcttgggtctatggctgaggcaaggggcttcctggcccgtgcagctgctgtgccgaggaggtagcacttctagtaacagcagctgacagcagggtgcaagctgccagcctctttccaaacggagctttgggggttgcagagcccccaaaggcagctgtgagtctaggtgttaggtctctcctgaatgtgatctgattggtcagttgcttctgcatctgtcttgaagacctccgctatcttgacgtaacaacgctatgcgagggggggaggggagatgaaagaaggaaggctgagggaaacccaaaaccgggagagatcaaagagcaaggtctacattgaaactaagagggctttgcgctctccatactgaagctgtttacatacaagaaagccagttggttgctatgagctttgccaagattataaagccagccctctagaatgccctgctttgggactcctggcacatcctcagctcctgaattgagggtcatcttgaatcagatcaccaatctctggtcaactctagtacatgacacatttgtctttggtcttacttaatccttgtcgcgcctgcatgctcggagttcttccttttgtttctgtcccgcaatggtgcttgggagagcattatccccaggtgcgcattcatatctgggtgtttgagtgtgcacggaggtcagaggtcatcctcaggtgtttgcttcccatcagttggactaggttgcttagacagagatcatcaggggcctacctggtgggctcccctccatcaccgggaatacaagcccgtacctggctttttatgtaggtgatggtgctcgatgtcaggtcctcacgtcgcacagctgacactttcctgaaccatcttcatgacagccctcccttcaacttgatttcccccccccagtagtactttttgaattactgtcatggaatccaaagaggtttgtagatcctaatggctcacctctaggaagtgtccacaaacaggcttagtgtgaaacccgtacccagatatagaaatgccaaatgagtagtaggattgattgtctgttggaaaaacaggctgtaacggaaacagcctgctacttctggctaacatttcttggtcgggcagagggcattgcagtgcttctgtgtgagacctggagctccaccctcagccctgcagacacacggggaaactaaacattccttgaccggctctcttgtgatcagcactgggagccgcttcagggaactgaacgggataaaatgcagctggggcctgagacctaattgctcagttgtagaaacaaatgctagcatacagagccaccagagaccaagaaaatactagactgcacagtcgccaccatctaggggagagtgtccctagggggtggggggaatgtgaacttgtctctctctctctctctctctctctctctctctctctctctgtgtgtgtgtgtgtgtgtgtgtgtgtgtgtgtgtgtgttcaatttgttgctacctctaaggccccacccctgacagtatttcctctttctgattgttccctcaggtgctcctggctctgctgatggggatacatccatcaggggtcactggactagtcccttctcttggtgaccgggagaagagggatagcttgtgtccccaaggaaagtatgtccattctaagaacaattccatctgctgcaccaagtgccacaaaggtaggagaaagtgagagcagagaattgtcttgagatttcttttgctttttttttttttttttttttgagacagggtttctctatacccctgtctgtcctggaactcactttgtagaccaggctggcctcgaacacagaaatctgcctgcctctgcctcccgagtgctgggattaaaggcgtgcgcctccacgccccggcttcttttgcttgtttctgatgttccccgaccttggtccctgggagtccccttattttgctgccccactccctgcccccgacttgggttttgccctttagttctccactacagcctgaccctaaccctatctacaggaacctacttggtgagtgactgtccgagcccagggcgggatacagtctgcagggagtgtgaaaagggcacctttacggcttcccagaattacctcaggcagtgtctcagttgcaagacatgtcggaaaggtaagccttgggattgggccagggctatagaaggtgcatggtgtgtgaagacgtgcgaacatgtgtgtgtgtccgtgggtgttggccaggaggtcaggatttcgaatctgctcgtgagtgtggcggtagtatgcatgcgtgcacatgcaagctcgggcctgtgtgcgtaggaggagtgtctgttacaaagacgaatgccatgtggcagagccagggggcgtcaagatttgtgtgggaaaagggatgtgagactcacacaccatttccttccctcttcagaaatgtcccaggtggagatctctccttgccaagctgacaaggacacggtgtgtggctgtaaggagaaccagttccaacgctacctgagtgagacacacttccagtgcgtggactgcagcccctgcttcaacggcaccgtgacaatcccctgtgagcaccggtcacccaagtcctctcccctccccgggagcaccctgcccccctcctctgccccccaccctatcctgtctgtgtgtctgagctcctatgtggcacctgcattcccgccctcgtccctccctcgggccctcagactgcaggcacgcgctcttagtcttaaccgctttcccacaggtaaggagactcagaacaccgtgtgtaactgccatgcagggttctttctgagagaaagtgagtgcgtcccttgcagccagtgagtatctgccaagtgcttggggttcaggggtgggtgagcagctgtggctgaggggccccagcagggtcaaaggtgggatcctacagccggatgagcagaagacactacaagacatcagacagccctttccctttctccaggacgttaggggataagcaatagggcttagcgggtaaagcgcttgcagcaaacgtctggcaacctgagttcaagctctggaaccccgtcttgtaaaggtgacaggagagaatatcaggtgcacaacgtcatcctctgactgccacacacacgtgctatagctcgcatgcctcttcagtgctgggcagttagatccgagcgcgctgttcttgactgcactctggtgcatcttactgttgatggtatcttaggtttggctcgcacaagctctaccgctggggatcccttcttcccaggctccctgacagacttcctcattcctgtggctccgcatgggctgctcttatacatttgcttccagagaagactctcatagttgacctgacttgggggttaaatcccaacttacctttttcctggctctgcaaccttgggcaagttcttacctctctacgccttatgtttcttaacctttagggtaaggagagtgggggtggagatgtggatcaacggtagagcactggcctagcgtattggaggctctgggttagatccccaaaacagacagctaaaccaacaatctataggactgtctgaaccaaagctgtctactttctatttttttttccacgcagtttcatctcaaaagagctcatgtgcccatgtgttcaccctgtcatgaggtagacaaaacctcctttccctgttctgctgagaacgcatgttcctctgccgtccccctgcccccacccagtgtagttttctcatcccctctgccctgtgacagctctcaatggctgccccaatgagagacatcctaaaacctcccgtgcccttgaggcctgccgtctccaaagtcaagtgctgtaagcagccggaccattggctgggaagccctccagcgtctcatatgagtcctctttctgggcacgcggcttcatcagcttaaagcaaagaccggctggtttcattcagctcctggtggttggcgttgctgctttagagtcagtgctgaggcaggggcatcatgatcagagcatactgtgcaagcacagtagctcacctcgcagcccctgagaggccaaaggaaagggtgtggagaggggtcaaaagtgagccctcagggacctaacttatactagtccccatgtcccagtatgctgggaccaagccttcaacacatggacccagcaggacatttcagatccatgccctaccggcaaacacaatgataaacccagtctactacagctgccgtctaccgtgccatgtcagggccaagtacttgatcccagaaggaggtgtcatgagcgccatgagatgctggaccagaaaagtgaagtgacttatttctgtcatgttgccagtcaatgactggaatggaatttttactcttgactataaaggccttttaaattttatttttaaaatactgattgattgttgaatccgggctcttcgcatgctattcacgtgctctaccatggagccaaaataccctcagcccttcgaccgtttgattttatttcatttcattttatttatttctttttactcagggtctcactgagtagccttggctggcctgggactaggtggaccaggctggccttgaactcctaaatatctgcctgctttagcctcccgaccactgggatgtgtcaccatgcctggcatttaaaaaatactttaagaattatttattttcattctatgtgtatgagtgttttgccagcatgcatatatgtgtactgtgtacattgctcagtatcctcagaggccagaagagggcgttagataccctggaactggagttacagatggccgtgagctgccatgtggggtgatgactgtgtcaaactcatcaagatggccgacttgccctctctctccctttcccctccctttcctctctagtctctttctggacaggatctcctgttgcccaggctgaccctgaccttgctgggtagccatgggtggccttaaaccgatcctttcgtcacttcctgccaagtgctgagatcacgtgcatccacttctgctcctgcctgtccacacagccttcccgggctcccatcagcttgtaaactgttgtacggtgtggactgtctcgttcttccccaccagctctcaaggcgggttgaagagatagcaaaaccatttgcaaagcaaagaactgcaggcagccttcctgctaaccggtgccttctcttctttcagctgcaagaaaaatgaggagtgtatgaagttgtgcctacctcctccgcttgcaaatgtcacaaacccccaggactcaggtgagggggggtggcttggtgccagctcaccgagctggctggctgactccatgacctccctccacccccaccctttaccccccagccccctagtctctgctgtggcctcacactgagcaacctctctggtctgcaggtactgcggtgctgttgcccctggttatcttgctaggtctttgccttctatcctttatcttcatcagtttaatgtgccgatatccccggtggaggcccgaagtctactccatcagtaagtaggactttggggatatagggtgttggtggagatacgggaggggttcgggtgggcaagttggagggaaatgaggggtggcctctcttcatggttaaggactctaggctgagtggccctggatggtgggagggaagccatactgatatccgtaattctcttgtccctggggccacatagaccctggggcatgacaccacaagtccccaaggtcagcgttgaaagggaagtgaaattcatgacaccttgtttctttgttctccagtttgtagggatcccgtgcctgtcaaagaggtgagaagggacgactccagcttccctgactactccttccaacgcctgatacctaaattacttggaatgagggcggtgggctcccttagctcctctgtccccacccccataaagaataaagcgcccgaagggagtccttttctttactcccactaatgctatgctttctttctttcaggagaaggctggaaagcccctaactccagccccctccccagccttcagccccacctccggcttcaaccccactctgggcttcagcaccccaggctttagttctcctgtctccagtacccccatcagccccatcttcggtcctagtaactggcacttcatgccacctgtcagtgaggtagtcccaacccagggagctgaccctctgctctacgaatcactctgctccgtgccagcccccacctctgttcagaaatgggaagactccgcccacccgcaacgtcctgacagtgagttgggttcctgctggggcattactcctggagggagtcgggcagggtggagggcacaaaggcaggctgctgctggaagtgcacggtccttgtccccagatgcagaccttgcgattctgtatgctgtggtggatggcgtgcctccagcgcgctggaaggagttcatgcgtttcatggggctgagcgagcacgagatcgagaggctggagatgcagaacgggcgctgcctgcgcgaggctcagtacagcatgctggaagcctggcggcgccgcacgccgcgccacgaggacacgctggaagtagtgggcctcgtgctttccaagatgaacctggctgggtgcctggagaatatcctcgaggctctgagaaatcccgccccctcgtccacgacccgcctcccgcgataaagccacacccacaaccttaggaagagggacttgaacttcaaggaccattctgctagatgccctactccctgtgggtgaaaagtgggcaaaggtctctaaggggaaggctcgagctggtagccacttccttggtgctaccaacttggtgtacatagcttttctcagccgccgaggactgcctgagccagccacttgtgagtggcagggagatgtaccatcagctcctggccagctgagggtgccaaagacaggattgtagaggaaaggcacaatgtatctggtgcccacttgggatgcacagggcccaagccaagcttctcagggcctcctcagtgggtttctgggcctttttcacttttgataagcaatctttgtatcaattatatcacactaatggatgaactgtgtaaggtaaggacaagcatagaaaggcggggtctccagctggagccctcgactcttgtaaatacactaaacgtctaaaaatga

SEQ ID NO: 10 - DNA, 2186 bp, Mus musculus
  source 1..2186: mol_type = genomic DNA
cgctcttgcaacaccacccccgccactctcccttcccctcctaccttctctctcccctcagcttaaattttctccgagttttccgaactctggctcatgatcgggcctactgggtgcgaggtcctggaggaccgtaccctgatctctatctgcctctgactttcagcttctcgaactcgaggcccaggctgccatcgcccgggccacctggtccgatcatcttacttcattcacgagcgttgtcaattgctgccctgtccccagccccaatgggggagtgagaggccactgccggccggacatgggtctccccaccgtgcctggcctgctgctgtcactggtgctcctggctctgctgatggggatacatccatcaggggtcactggactagtcccttctcttggtgaccgggagaagagggatagcttgtgtccccaaggaaagtatgtccattctaagaacaattccatctgctgcaccaagtgccacaaaggaacctacttggtgagtgactgtccgagcccagggcgggatacagtctgcagggagtgtgaaaagggcacctttacggcttcccagaattacctcaggcagtgtctcagttgcaagacatgtcggaaagaaatgtcccaggtggagatctctccttgccaagctgacaaggacacggtgtgtggctgtaaggagaaccagttccaacgctacctgagtgagacacacttccagtgcgtggactgcagcccctgcttcaacggcaccgtgacaatcccctgtaaggagactcagaacaccgtgtgtaactgccatgcagggttctttctgagagaaagtgagtgcgtcccttgcagccactgcaagaaaaatgaggagtgtatgaagttgtgcctacctcctccgcttgcaaatgtcacaaacccccaggactcaggtactgcggtgctgttgcccctggttatcttgctaggtctttgccttctatcctttatcttcatcagtttaatgtgccgatatccccggtggaggcccgaagtctactccatcatttgtagggatcccgtgcctgtcaaagaggagaaggctggaaagcccctaactccagccccctccccagccttcagccccacctccggcttcaaccccactctgggcttcagcaccccaggctttagttctcctgtctccagtacccccatcagccccatcttcggtcctagtaactggcacttcatgccacctgtcagtgaggtagtcccaacccagggagctgaccctctgctctacgaatcactctgctccgtgccagcccccacctctgttcagaaatgggaagactccgcccacccgcaacgtcctgacaatgcagaccttgcgattctgtatgctgtggtggatggcgtgcctccagcgcgctggaaggagttcatgcgtttcatggggctgagcgagcacgagatcgagaggctggagatgcagaacgggcgctgcctgcgcgaggctcagtacagcatgctggaagcctggcggcgccgcacgccgcgccacgaggacacgctggaagtagtgggcctcgtgctttccaagatgaacctggctgggtgcctggagaatatcctcgaggctctgagaaatcccgccccctcgtccacgacccgcctcccgcgataaagccacacccacaaccttaggaagagggacttgaacttcaaggaccattctgctagatgccctactccctgtgggtgaaaagtgggcaaaggtctctaaggggaaggctcgagctggtagccacttccttggtgctaccaacttggtgtacatagcttttctcagccgccgaggactgcctgagccagccacttgtgagtggcagggagatgtaccatcagctcctggccagctgagggtgccaaagacaggattgtagaggaaaggcacaatgtatctggtgcccacttgggatgcacagggcccaagccaagcttctcagggcctcctcagtgggtttctgggcctttttcacttttgataagcaatctttgtatcaattatatcacactaatggatgaactgtgtaaggtaaggacaagcatagaaaggcggggtctccagctggagccctcgactcttgtaaatacactaaacgtctaaaaatgaaaaaaaaaaaaaaaaaaaaaaaaaaaaaaaa

SEQ ID NO: 11 - protein, 454 aa, Mus musculus
MGLPTVPGLLLSLVLLALLMGIHPSGVTGLVPSLGDREKRDSLCPQGKYVHSKNNSICCTKCHKGTYLVSDCPSPGRDTVCRECEKGTFTASQNYLRQCLSCKTCRKEMSQVEISPCQADKDTVCGCKENQFQRYLSETHFQCVDCSPCFNGTVTIPCKETQNTVCNCHAGFFLRESECVPCSHCKKNEECMKLCLPPPLANVTNPQDSGTAVLLPLVILLGLCLLSFIFISLMCRYPRWRPEVYSIICRDPVPVKEEKAGKPLTPAPSPAFSPTSGFNPTLGFSTPGFSSPVSSTPISPIFGPSNWHFMPPVSEVVPTQGADPLLYESLCSVPAPTSVQKWEDSAHPQRPDNADLAILYAVVDGVPPARWKEFMRFMGLSEHEIERLEMQNGRCLREAQYSMLEAWRRRTPRHEDTLEVVGLVLSKMNLAGCLENILEALRNPAPSSTTRLPR

SEQ ID NO: 12 - DNA, 42218 bp, Homo sapiens
  source 1..42218: mol_type = genomic DNA
gcgagcgcagcggagcctggagagaaggcgctgggctgcgagggcgcgagggcgcgagggcagggggcaaccggaccccgcccgcacccatggcgcccgtcgccgtctgggccgcgctggccgtcggactggagctctgggctgcggcgcacgccttgcccgcccaggtgggtgactcgcgcggcccacgggggacagccgccccgcatgtccacccggctggtgcgcagccttcgggtgcccgggccgcgctctcccggggcgctgtcacgggctgggaggctgggagtcccagtcgccgccccccatccgcatcagacacgcgcgcctctggggacccgctggggactccgggcccggcacacgtgcgctcggggcacaactctggcccccgaagcccctcttacccgcgtcgtgacaggggcgcaccctggttcctccgcgagcgcaggccggggcatttggggctgagcagcgggtcctgggcagacccccgctagacccgggacccctcttccctcaccccggcgactgccgcgacagcccttccctcccacgcggtggagaaggggctgtgccggggcgctgccccactgcccacgccgggcaccctcttcaaaagacttccttttcctctgggcgacggttttccgatttcttagaaataccagggtcctgtgtctgaagagcaggaccaggtgtgtgtcaggtccactgagggcacagctggagggcgagctgcctgtctgcttcctccgatgcgtccgggggctactgcagagtctgttttctgcggcctctggggacagggcaagcgagggaggtctgggctggtaatcgagcaaggcaaatgaagtctccgggggccgcaggaaaatggagacagcagaaaccctagggctcctattcaatatgaacgtcactcccacagtagcaacgggcgtacaagggactgtgcaccctttgcctgtttttgactgtctcctggtctggtaacataggataaccccatttttgttttactgtctccatggtttggtaagataagataaaccattttttagagaaggaaaactgaggctcagagaacttgtatttcatggaagggtctggggggaactcttcctccaaagggggcctctcctgccttcggcccctgtgccctgaggctgcggggaaggtgggcgttcatccttcctcagagccgcccctgatggacacatggcccatctgcccccatctgacatcttgaccgaggaggaaggtgggaggtggcactggcttctgtggtgacataaggtgacttgttgatctgaggccagagagtccagttcttgtgggtggaagatgggggctgtcagactagaattgactcaccgacagtgggtgtcaggagtgggtcctggagaactgccccagagtaagtcctgggtggcctttgggtcaggagagtccccactctagggccgagtgtgaatggggacgaccgtggtccccagcttgactttggggtcatgccatatactctggcctcagagggggtcttcctgccgctgagcttgggcctgcctgggtgaactctggggtcatgtgagcccctggatgggagaggggtgtcaggcacagggctcagcaggacaccaggctgcagtcctggagtagctggaggaggttccctcccacttccttcccttcctgaccagctcctgcggcagctcatattccctcctccctcatccctgctccccacgaccccacccggactattgccgcagccttgtagctggtctcccggccctgccccctctcccgctgatccttggcagagagacccttctcaagcatgaggcacctctctgtttgcctggggagcctcctgtggctcccaatggttgaggcagaaactcccctggagatcccaggccagagtaaggtacctgaactcttcctcgcgcctccctgcacatgtgctcccccgcctctgtagaactgatgatggtcatcgtgtgtgtcattgtgcaaaaagcattgtccgtgccatcccctctccaagggacacttcttacccctatccttcaaggccttctgcaaatgccattctctccaggaaagcctttccgcattctcagttggatttgatcttctcttcgaactcccaggcccttttgttccctttgaggacagattgcattctgctttttaatctagctgtgttttatccccctcagtggatggaaggtgtcttcagggccagaactgtgggttcctcttccttctcatcagtagcatcgccatagctcctgatttctgaacacccactaaacaccaggcactgggctaggtactttgtcacaaaatttcactgaaacctcccttacagcaactcccaagaggtgggtggtgccgtttgtctttagagatgtggaaactgaggcgtttcccaggatcacagagctgggggccggggagctgggggtgggatttgaatgcaggtctgcctgattcccaagctcctttcactgcaccctccccgtgcccgtatctgcactcatgctcccagccaggccctcacacacagtgggttctcaggatggaagtcaactgagctgcagaagaagcccccaggagacctgagctagccatggacgcagccgactcactgccagcagggcttttgccccgtttaaaagtcttatttgccagctggtatggaaaacatcattcattcatttagccatttattcatttgacaaagaaatgccagtaaacctggcagtaggtgagtgcttggtgccctctgatggggatgagcagggtctgggctgtctggggaggaggatgaggggtctctgcctgatgggcctggcccacctacccctggaagtcttggtgctgaggtgccactatttgcctcctcatcacccagggcctggggccagtttgggttaggggagaggttgggggctcccaggctggatgtcaaagaggagttgggtgatctggggtacctgctggccctgggggctcttccctccttccaccacgtctctgtctctttgccctctgtctgaaatcccagtggggaccctgtgtgttgactgagggtgtggtctgttggtcaggcacgtcttcagagggcaatgggtaggtggccaggcaccctgaggcagggccattcattcattcattcattccccaaagttcatggacacacctagtccaagcccagcccagtgcctggctctggggacctcaagatgactccagctccaatcctctaggagctacactaccaataggtcacagacctcacagacctgggctctgtcccaactgcccttatgagcttagctgagctagtaagcctatgttctcatctgtggttgtggaaagtattccctgcctggcctttgtcacagagccatgggtgtgaaaggctgagaacctgccgggcattcttacgtcagaggtgaccctgccatcctggcacctggcacagtggctccccgtagcactgtccctccccacggctgggtgacgctttatggtccttactatgcaatgttttctggaggagtagcagggacggttgtgcgtgggaaggggaagagttttgccggagccatggcatgtatgttacacccgactctacaccaactcacttcttactttttttctgagatggagtcttgctctgttgctcaggctggagtgcagtggcgacatctctgctcactgcagtctccatctgcctcttgggttcaaacgattctcctgcctcagcctccagagtagctgggactacaggcatgcaccaccatgcccaactaattttttttttttttgtatttttagtagagtcggggtttcaccatattgcccaggatggtcttggacccctgacctcaagtgatcctcccgcctcagcctcccaaagtgctgggattacaagcatgtgccactgtgcctggcccgttctcacttcttcttctttttttctatttaatttttttttattgagatagagtcttactctgtcacccaggctggagtgcagtggcccaatctctgctcactgcaacctccacctcctgggttcaagcaattttcccacctcagcctcccaagtagctgggattacaggtgtgtgccaccatgcccggctaatttttcctttttttttttttttttagtagagaccgggttttgccatgttggccaggctggtctcgaactcctgaactcaagtgatccacctgcctcggcctcccgaagtgctgggattataggcgtgagccaccccacccagccccattctcacttttaagccatgcttttctgtcctcagatgtgctgcacacacacctgctccagggcctttgcacttgctttccccatcacctccaatactcctcctgctgacgtctcttggtctccttccctcgcttccttctgctgaagtagacaatcctgcctgtaggtgctccctgccaggcactctcactccctgacctgctttgtattcctgtataatgctcttgacctattctatttatttcacttttattatgtcttcccacaagattgtaagtaccgtgaggacagggactcattcaccactgtagactctagcctagaagagggtttttcagtcagtgcctctgactttaattctttgttgtggggctgtcccgtgagctgtaggatgtttagcgacatccctggcctctacttattggatggcagtagcgccaccctccctcgtgacaaaaatatctccagatattgctaagtgtcctttggggttgggggattgcccctgattgagaaccactggcctaggacagtgcctggcacatagtaagtgttcaaaaaatattcatctgaccttgaccttgataatggccctgttttacagatgagacgggggtttgaaaagtcagtggtggcagggtggggttctgtttgcctccatctcttggggtatttttctgggctcctcttcccattgagtggtgtctgctgaggttaggggtcctctccccaaattgctcaccccctcgacatccctcgtgtagtgagggatggggccactcactgacggtgactcagggccccagaatgcatgtgatttacccagaagcgggcaaggagggaagctggggtttggggtgccggggatgaacaggaacaaaggagaggcgctgtggctccccgttctggaccctcgtctggccacagggaagcagcactgatgactctggggaaaggccccggcctctgaatcagataaacctcaagtcgctgctctgctgttttactggctgtgtgacctgggcaagtctttctatccctcggagcctctgtgttcttatctgtaaaatgggagtaatcctagcctcacgggctggctgtcaggattaaaagtgctttctaatcctggcattggcagctatttgagccattggtggctttgcaggtctgacccgactctctgggccatggggtggtgctcgggcctaggtggggacccctgtggagtcagactgtctgctctgagccccagggccctgaagcttgggtggcagccctgcagttgcccagagttcctgtctaagtggctttgttgcccatcatctcagaaagcaacttctttcctccctgccttttcctgtctgtgcttctgccccagtgccccctggctgggctctcaaacccactgcttgacagcctggtcttaggacactgtattgtggcaaaggctgtggggtcaggatatcccctcccctccctttgccaccccttttagtgagtaacaggtgctgtgtgttttggggatgagtgaagggtacatttggtgaagcacagagagagtgcacaaggcttcagtttgcaagatgggcacgggaagattccaggccatctccaaaacctcttccatctccaacctctgtgctgctgaaggttctgtttacttgtgaccctgagaaggggatgccctatgggggctcttctgagatcatgctgtccattttcctgcctccaagtgacttctaagacagcatggctctgaggaaggagcactgacttgggtgttgggagatcacagttcccatctgagcaccgtcactggcttgctgtgctaccttgcttgggttacttaacctctctgggcctaagcatccctatctatgaaacctaacaaccctggttccaatgctttcctagaatattggggaagtgtcggctttgagtatacttgacaaaggccacagattgggggtggggtatataaaagtctacaggaaggagagcccaggactccccactgtcaatatcttggttccccagcttctcttcttcttgctgacctcaatctcacttgctttgggtggattgatttcctgactcaggctccagggccatcaagaattcacggctgcctttcagccttcatgaaggacatggtggagctccttaggcagaactggggtttgtggatgtcctgcctctctgccccttggtacctaggtggcaccttttcaagttcgggagctagatcctttccccttccccacactgtaggaaagtccttactgtaggcaggcgctgcagagcctgctgtctgggaacccacaggttcaaggaagccttgagcaggaagggcgttttcctggaagaagccctttgtcgctggtaatgggtgcaggctgctctgacccggttctgagtcctgcccccttccaggcctagggctttgggccttgatcacctctgctgagtagctgactgcggggctggggctctgatgctcaggacccacctctctgggacccacagtctttttccactgtggcgtgtagtgatgtcacaggtggcagtgatgtcactgtggtttgaggtacttggctgtgagccccggaggaggaagtgtctgttcgctgatggggggttggaagagatcattgacttctgccccaagcgtgagccccaagtgtgcaggggggagtgcggggggagggctgttggcggcgcatcccagggctctggctctgcccttgcatctagcctgtctttcctgtgggctgtgacaagccactctgcatctctgagactccatttcttcttcttcttcttcttcttcttcttcttcttcttcttctccttctccttctccttctccttctccttctccttctccttctccttctccttctccttctccttctccttctccttctccttctccttctccttcttcttctgatggagtctgactccgttgcccaggctggagtgcagtggcgtgatcttggctcactgcaacctctgcctcccaggttcaagctattctccagcctcaaccttccaagtaactgggattacaggcatgcaccaccacacccggctagtttttgtatttttagtagagatggggtttcaccatgttggccaggctggtctcgaactcctgacctcaagtgatctgcccgccttggcctcccaaagtgctggaattacaggcgtgagccactgcgcccagcttccatttcttctttgaaaagtaggaggggttggaattgtcaccctggaggttcatggttgctagattattgattctgttgctggattcaggagacctgttagctggctagttcacagcaagtattgggtgtttggaggggggctgcagagccccttctcaggccccaggagggccagctgccctccctaccccctcttttggacactagtgggcatgttctgctgggaaaacagacagtgtaacctgacttcgagggctgcaggctgaatctctttcagatgtactggctccttgagaggcctagcagatctctactctgtgggtccctttcggagctggggctcaggtttgacccagccactctgaccggagacagcgcagaaatcaccaggagcatttgtttgttttcctttgctgtccagacagtggcccaccgtctgcttcagtctgagcgtggccctgcactagtgagactgatgtggccacaggttcagagaatcagtgcgcctgagtgggagagcagagcgggaggggatttggaggcaggcgggctgtggacagggaggggggaggacatcttccgagctgtcagcgggaggccttcttgaaggtctttcaggagcaaggccagaggccgtgggagtgggcggggcctggggctgggagtcaggggtctgaggcctcatcttggcccggcctctgcttccgggagaacttggccaattcccttctcctttctgaaccttggtggccccagctgtcacttgagattagcaaggacctccctggtcccagcaggagtgagtggctttgggcagggggtggagtgcagattgcactgccacgtcacccagctcagaaggcccaggtgtggtccagctgtggacttgattgtgaactcctggggaagggctctggtcctttgcctcagttagcgggacccccaccagtgccctgggtgcccctgctggcccctcctctcgctgaccccagccccagtttctggctgcaactcacagaggccccaggctcctgtggccccatcaccagcagctcctgctgtcatttcctgagcctcgcaagcccctaatcctgctccttcctgtcctggcccccagctccctcaagccccactcctgcatcccattctccctggacatcacccctcccaccccttggctcaatttccttcctgtcgtggcttggtcctttggtcattgccctggtcttttcttgtccccttcctgattctgcccttctccaggcccacacggggaacctcctaaccgctgagccctgaaaggtaggcgggtttaggatgagtggctacagggaggagaatggtgtggggagagagatatggaggaaagaatattaggggacaggccgggcacggtggctcacgcctgtaatcccagcactttgggaggccaaggcgggcggatcacttgaggtcaggagttggagaccaccctggccaacatggtgaaaccctgtctctactgaaaaaaaaaaaaaaaattagccaggcgtggtggtgtgcacctgtagtcccagctacttgggaggctgaggtatgagaatcacttgaaccccagaggcggaggttgccgtgagctgagatcgcaccattgcactccagtctgggtgacagaacgagaccctgtctcaaaaaagcaaaacaaaacaaaacaaaaaccgaatattagaggacaatgttaggactgtcccagctgtcctagctggagccaaaggtttgttggggacagtgacagcagcacacgaggctgtaagtttagggccagtttatggaggagtagtaccaattacattgagaaaactgtagcaactataatttgggaggaattttctaaatactttacatgtgttatttaatcttcccatcagccccaggaggtatgtgcatttatcagtcccattctacagatgaaaagactgaggtctatgaactcctttatttaaaaacaaaacaaaaccccctcaaggctgcctgctaagaggggaggagtgtggattcaagccagcatccttattccagtgtccatgctctcagccaccacacacacactcctatcaggagttggggcagtggggagccattatagtttttgagcaagagagtgacagggcaaagatcactgtggcctcagtgtgaagcacagatgagatggagagactggaggcagggaggcccatgaggaggctgtcaacatggttcaggtgacagctctgggttggtgaagaagcagagaacaggaaggaaggggcgagaggcttgagggaggaggaggaagcctttggactgggccgtggatatagggtgggaacataggaggtgaggagcatgctctctccacctgctttttgcaacatgcggcctctctggccttagctctgcctgtcctgagccctgagccctgagcccaatggaccgattctgttttttttttgagatggagtcttgctcttgttgcctaggctggagtgcagtggtgtgatcttggctcactgcaacctctgccttctgagttcaagcgattctcccacctcagcctcccaagtagctgggactacaggcgtgccccaccacgcctggctaattttttgtattttttttagtagagatggtgtttcgccatgttggcccggctggtcttgaactcctgacctcaggtgatccacctgccttggcctcccagagtgctgggattacaggcgggagccaccgtgcccggccccagtggactgattctggtcagtgtcaaccccatttgtccctggagcttttgcagtcggtcacagggccagcccggtcctggtcaccgctggctggttaccccggctgggttgggcaggagtctgggcagggctggttgctcatctcaggtatgaaattggctgcacccccactagtgtgggggagcaggattccagggcctgcctggcgctgctacccctgtgcctccagacccctcgagctcctcccagacctttggcttcgttgactgtgaggtgaaaacaaaagggctgctctctgtcacttcccctaggggcgggcagatgctggcagggcacagagagccgagggctaagagctgacatttagcctggctactcaggagactgaggcaggagaatcgcttgaacctgggaggcggagtttgcagtgaaccgagatcgcgccattgcactccagcctgggtgacagggtgagattctgtctccaaaaaaaaaaaaaaaagaagagctgacatttagcgggtgcttcttgggtgcaatgcgcaagagaccgatgcattaactacacagagtgcccttccttgtcacagctacctgggggcaggggaacatcatccccattttacagaagaggcctttgaagcacagagattaactgacgtacttagggttttgcagctcactagaggcagagccaagactccaccccaggtggccaggctcctgagcgctatgcctacctcaccctccaatgaggtggtggtggaggagaccgtgagccgctgtcacctgaacactggtgcactcagtctgctgctctgaggacgccgccccctctctttgtaagtccatttcctgcccatttctcatgctagctccagctcatttcaactaattgaaaattaaaactttgcttctgttgagcaattcggcatcgatgagacgccagctgtgggctgtgtgctggctgtgtgtagggtgatgagtagcagaagcacgggtgacactgagctctttccactgccgggcacggtgccaagcacgccacgtatactgacttcatgaatcataaagccctgtgaagggggcactgtttctgtcgccattttatagatgataaagtggaggtgggggaatggcagaactgggatcaaagcccacgtgtctgtgtctggctcagcgcccatacaagggtgtcaaggttgcggggaggcacgagggaaccaataattaaccaaaactggtcgggtgtgggcagtatagagatgcacccgggttgtcacaggagcccctaggagggacctctgacctccctgaaatgatggcagagggaactcttgaaagaagctgagaagtcagcactgccaggtcgggggtggcgggtcaggacgtttgggcagaggcagcagcagtacgggcatggagaagggggcggaggagccaggtgctgctttgtgttgtgacagcaacaggtgagtgatgaatacaggtgggagatgctggcaggggctaaggaggttgcgcaggtggtggcagccgctggaagcttttaaggagagtcaggcttgattgtaggaagggggcttaggtccatctgaaagggacagaaggctgggaaccaagaccaaggagcctgcagctggcaggagatgctgagggcagcgaggaggaggggtcgtgggagatggagcaggcgacatcagcaggccccttggagggtgacggtgggagaggctggggcgtctctcattagactcagggttccttgcaggcagggaccatgcccggcgtctttgtaccctggcatttagcacaaagcctggctccaagaaccggataccagcccagtcttcctgtctgcccccagctcatttctaaagcaacatcacaggcagcgagtcgggagtgggatgtgtcacccccgggttgcctgcctgtgatgtggtcagtccttcctaacgcagatgccattcctctccgtgacggcagacgggcctccgctgtcactggccctggcgttgctgtgacgacctggcctgatgtagctgcaccctgcagtccatggggctcctgtgaacccccaaggttgagacccaaatgcctctgctgcctcccaccacgccctaggggccccgcgacccgccatgcaaatgacgtggtttccgcattgcttgaagagggtttcctctgtgtgggggtccctgggtccttgggcagatacctctgcccctccccacagctttggcccctgccctaagaccctggagacccttttgcctgggagagtcactgaaccacctgcccctgctcacagtgtgttcacagaagagtcactcccctctgtgggctccttgtctgtaaaatgagggagcaggacaagatcacagggtacaaaactgtcagagggcacagaggctgatgttgctgccatcagctcctggagtgccgctcactggctgcatgaccttggacaatttgcacgaaatctcccaagcctcaatgtctgcatctgtaaaatggatcatcctgacctcattgcgttagtgctaggataaaataaagagaaggtatatgaacgtgcccagcactgtgcctgcacacagtaggtacttttcctggatctgaacagtctctgttcttccagctctgtgtaaaggcttgatctcgacccctaaagcctgaagcttctccctgtggccacctccccaccgcatcatcttccgttctcagcgggtagatccctgcccaggggggaccccctggggaaggctgggagcatgacctcttcccaagggtacggcatctaaaagggatctccggaacattgaaaagccatgaaggccgggcacagcggctcacgcctgtaatcccagcactttgggaggctgagggaggaggatcgcttaaggccaggagttcaagaccagtctggacaacatagcaagacccggtctctttctataaatgaaaaaataataataaagccatgaagatccccaaagaaggctgtgctaatggcggccggaagagcagagggcaccacagatgccgtgctttcagctttttccttctcctccaggcctcccttctttccttcctctctcgctatttataaataagagaaggcattgagggcccccacctcgggtacttgcagggccttggcctgggaacaggacaagcagcaagtcagttgacccggggttgctcaattccccaagagctgacgcaaactccagaatcagacctgccctggccacctggccctgccccttaccagctaagggctccagcagagtcctagtcttgagcgaatcttatacctgcagccctgtccaccagctgtgcttcctgagtcctccagggtgagggggcgtggggtcagaagagaggggacggtgtgcagggagggtggaacctgactgaccgggtcagccttactcttccagcggggtcttttcttcctggagctcggccctcggcagctctcagaagctcaccttcttgcaggctctcacagccgcatcgtcctctggctgggctgctcacagaccccggcccctgggttttgtccactcacccagactctgttttggggtcacattacccttccagtgttcctctgagcaaagtccctgtgagttagcccaaggtccctgtcaaggaggaccacatctggcctgttgcactcttctcctttgccccaccgaagcctctgtcacactgtcacagcagcgggcctgccatggtctccccatgtaaggcttcctgaggaacgggcctggtgccagcctgggggtgaactgccagccccaggagtcacaggtcagcttccccacacttaccctggaggcaggatggaggccccctcctttgcaaggcccacacgggccatctaacaccccactaaagccgggcagttcgctgccctggggtgtgttctcgccttgccagttcttggctaaaaccaaggcaggaagagcccagttcccatgttctgtaacatgggtctatgaccagggcctttgcaggccccttgcagcgcccccatggagcccccaggagtctgggagaagatgatgaacccaagtgaggacctccccaggggcctttgctcctcacaagaacccctggaggagacagggcaaggagtaccactcccattttacaggtgacaatgccgaggctcagagaaagtccatgacacccccaaatcccccggacccactaccctgacctcctggcggtgcacagagcatgccacgcacctctccatatgcacatagaccctctaacctaagtcagcgccccttctacaaggccggtgtccagcacacctgggaaaggggacatttctggccctttcctctcagaagtcgcctgctcgagctgccctccctggggggaaggggatgggggcagaagctgagcatggaagcccctgctaatccaccctctgctctctccagaggcccaggaccagcccaactctgccccacatcccagcccccacctcccagctcgtgctgtttctccacctctcatgtggatgggccacacaccacccagcacccctgaggtctggtgagggactgagccttcgacacccatccttaagaacccagggctggtccttttgcttagagcatcaaccaggcccacactctcattttacaggcagagaaactgaggcacagagaacctggttactgcccacagcagaggagacacttgagtgaggacacagaggatctttggggtaggggcgggccttggggttgagacccagtcttcctggccagggaggaaacacaggactggaggtgaggaggcctctttgaggctagtttcttcatctgtaacttgggaataacaataggactggcctcagggggaccaggggaggattcagagaggctatgatgctgggacagctcttcgtgatgactggcatgaagcaggcttctagtagatgctctactgctgctttcgttctcaccctcacccacccgctctgggcccactgccctgacctcctgaccaagcactgagtgtgccaagggcatctccctgtctccccggccccgcaccttgtgtcacccttttccttagctcttaccaccaccttgaattctctattgaacgtgcatgtgtctccccagctaagatgacaacttcccgggggcagggatttgatttgttcaatgctactgtttacccagcacctacaacactgggtgctcagcacgtctgttgaatgaatgaatgaatgaatcactgctttcacctttgcccctgactttctccatggaccacggacaagtgacttgatctccctgagctgtgaaatggggccattcacaccagctttttagggtggaactaggattttatacagtgcctgccatctggcctggcacatagtagttgcttagcaaatatcccattgttttccttcctccccagagggccaaagccaagacctggaggagcaacagggtgggggtctaacccctgggtgacagagacagctcccatctgggatggaggctgcatggtgggaggagctgctgaggttgggccattcagctttggggcccttggagtcctgggtctgtgtggagggggaagggaagctctctgggccccaagagaagggaggcaggattgggggtggcaaggattgcagctcttctgggatagccttgggcacactgctttgtctccctgagcacctgcgaatgtcagtgagaagaccagacagtgggtctaacacgcacagttgcccctgggaggtagcaggtgctcggtaccgatgagctaccgctaactgcaggtgctacctgtcttagaggagggagcccaatctggaggaggggaaatgggagctgtggacccagatgggaggcggctcagagactgtgggtgggccctgatgagcttcttatccatagtcctctatccgcttgccgccatcctggccctggcatggcccaaagtctctgggagacgaggggaggtggctttgcctttttccatctctgttatctcatctgtgaaatgggcacaatcagacctgcctcaccaattggaatatagatttaggtgcagttttcttttttctttccttttatctattctctctctctctctctctctctctctatgtatatatgtatagctatctattgatattttctatcatccatctatttatcttgtatctactttctattatctctatcatctatttatctaatctatcatctatctagctatctttctattttatctatctatctatctgtttgtctgtctgttttatctatctagctattttatctattttatctatctatctatctatctatctatctatctatctatctatctatctatctattctatctacctatctatctatctatctatctatctatctagctagctagctagctagctatctattctatctacctacctatctatctatctagctatctatctattctatctacctatctatctatctatctatctatctacctacctacctacctacatatctatccatcctctccgattccctcaccactgggtctcagattccctgcctgttaaataaatggtcagttaaccctcaacagtgattttcaatttttcacttgaggcccccatattttggaagattgtagtttgctgaacacgctgactgaatcaagtactatccaacttatttcctcattttaacatgtcaaagatcccctgtggggtgagtggggtgtgaattggagcctccccaatccaaggcacaggaactggaagcttctgtagccctgcatttcctagagaatgcttgccatgttttggggacctcctggggggcccctgtactgaccagaggccggctcccagggctgtggtttgggcccagccccctgctcctggggactgctgctgtggagggagtgaccttttgttctgctttgccaaggggctttctgttcctcattgtttagccatgacaaggctgtggatttttttttttttttctgtccaagagaataaacaggcctgagattgctcaagggagccgaccccctctgccagctactgggggctggaggctcacagagccagggaggaagtcctaccccctctgccggctaccgggggggctggagccacacagagccagggaggaagtccagggacggtcactcacagcaaagcctcagacaagagaggaacctggaggggaggaggtgggaggccaccactcagccggcctgggggccatgggagtccagctgcctgccgttagtggccaggagccctcgtccattgcggctcttgagagcccaaacttggccacggcagggctctttcccatcaggccctttgagccctgatgggaaacccttccccagccagggtgggatttcttgctgccgcctggagccgccctggccctgtggttctcaggccctggaggagtgaggggctcccctggttaccccaagggcactcgtggggatgaagcccgcgggatgcaggattcccacgagacctgtgctggccactgtgcggggtggggggctgccagggaagaggtgcagcccctgcctgcctcagggatgcgatctgagggaagaggcagctgtgtctgggaggccgttcggtcggagggggataggcacagcccctgcccttggggaagcgcccagcagcagccttcagggaaggcagtttgggggtttgccgagggccaggaagaccctctgccgcagttagtattcgatggaatggcttgtgcagagggagctgcagaagctgccatttctctgggttaggggctcccacagcctttggatgccgggtctcggccatgagccccctccgccacccctcccccaggtcaccttgctcaatccaggaggccggatgatcagagtgtgttctgcaaaggagcgtgagaatcactggggagatttcctttttctttttctttctctttttttaatggtacagcttcctgggcccacccctgagattctgcacttgtttggggagtgggtgttggcttcatgacaggcacccctgggtgctttggacacaggcagtgagctccccccacactgtgtgaacccctgagaaggcttctccttttgtctagggtgcctgggagtctgctccagcagcaaaccggggaggggaggggtactgggaccgagtgtgtgtggcagcaccgtgtccaggcaaactgaggctccagacgggggttacttcttcagaccctgttatgcagcatggttcccactgcccgtgcccagaattcaccatagctgatgggcctggggtgggcctccggggcaggccagggtggaaagtgcatctgtgtttgagctttgcggccctggcgctggagttagatccctacaggaaaggacattgtaacccagcccgtggttgagactagcagctgctgagcacctacgccctgctaggctgtggggcaacagcaaagggtaacccccagcctgcagcctcaggggggcttcccatctagcgaggggcccagggaggccatgaggagagccatgagggaggaaggtggggactctgggcctgagtgactccttcagggtggggtgcgggcagggagccttcaggagggagggtactgcctgagcagggctcttaagggacacgtggaatttgttacaggaagcaccaggccattccaggcatagaaatcagctggggtgcaaaggcctgggggtcagaagagtggcagattgctccatggcaggaagccccagctcctctgggtcgttcccgctgagggattccagctgttggcaccgaggggtgcagccagggcagggtggtgctgcctgccaggctgaggtgggagacagctgggtttctagccctgcttgtcactcgctataggtgcagccaaacgctcagcaggcccaaactctgggcagtcctgactcccaggcagtgctgtgaggaaggggaggaggaggcacactgaacccacctgctacgttggctggtggaaatttggccaggtctgcactggcccagcggtgctgggtgtcgtgactggtgtctgctctgactggcttgctgacagctgaagtccaggataggtccatggccacgttgtgctggtttgttaaatatttttagtatctcccctgctcctatatgttaggtactggagtccagagaggttaaggcacttgcctaaggccacacagccgctaagtggtggagtgaggatttgaaaccagttctttctgactccctgtatccttatctatggagaggccccatgactcgttcactaaaggttatggatctcgatcttgtactggccacatgactgcagctggcagtacagtggggagtgcgccagccctggctctgacctcctagaactgccctttgttcatttccaggtgacgcatctgtgggggcccctgaaggacttggggtgtgtgtgtacaccctctttgcttgtacagatgtgttcacacccatgtttgcctacatgtgaatgtctccattctgagcttgctctcagcctggtagaggtggctaattaatgcttgtccctgaaagcccggactgccaaccccagtctttcaggagagagggcaggactcaggggcttgctcccgggggtcctgggaaggcacaatggtgacagtgctgcagctctgcactcctggagggtcactcagagacccgagagaggagggctctgcgtctgctcctctgtccagggctgtagcttctctgggtgcctttgcttttctcttttctcccctctttttttttttttttcgagatggagttttgctctgtcaattaggctggaagtgcagtggcatgatctcagctcactgcaacctcctcctcccaggttcaggggattctcctgcctcagcctccagagtagctgggattacaggcacacgccactatgccgggataattttgtatttttagtagagacagggttttgccttgttggccaggctggtctcgaactcttgacctcaagtgatccacctgcttcggcctcccaaagtgctgggattacaggtgtgagccaccacacctggccctctctctcttttcattcatcacattgttcatctcttcccggaggcatccagcacagtctttgagactgtgagctgtgaagtcagacaggacccaggtccaaacccttctctgtcacttaccaggtctgggaccttgggcaggtgacctgccctctcaggcctcggtttcctgttctataaaatggctgcagtagggaaaccgtctccatcttcattgggtggttgggaagtcttgctgagaccacacacctgtctcaggtagggtcttccagaagcagagcctgaggcagggatctttgtgaaagtgatttgctagggagggctcccaggagaagcaggcagggcaggtcaggggagggggcttagcagggacgttgttcaccagcttcagcccaacaccacgggggtggctctggaccatgaattgtaccagggtgggtcccaccttgaggctgtggagcattcattatcagccaacacccacagcagctgggggagcggtgccctgctggcagcaggggtctgagtggggtgcaacagcacccaccaattcgagcagcagaaacgcttagaacagtgcctggtacctaggcagtgcttcaaaaatggcaacgattgtcatggtcataaccaacattcagctgatgagtgccggctctacggtgggtcccatgtgagagattgagggtctagagatgacaaggctgccacctctgctgtctgcatcacatgagtgtgtgtgtacacatgtgtgtgcatacatacccacagggggtggaaggacaagcaagtaaccattccagaacaatgagatgactgttagaggggtcataacccacgtttagagagagccgagaggaggaggaggaggagcttgaattagccttgggtagtcagggagggcttcccagaggtggcagcactcatcttgaaagacaaagggatgtttcaggtgcaggagggaaggagaggtatcttccttcctcagcagagggcagctttgtgctgagaacccccgttctctgtgaccaaggccactgtcttctggatatctgtcccatgcagtgttaggggtcacccagcactggagaaggccagcagagtcagtgcttctgcctgcagacatgactagggtacactgaggtggggaggcaggggaggtaaaagaaggcacgagctctccttcctgtaccctgctccagggggagaaacctccccagccatcatcagtgcagactggcagggggagggccaaacatttgcagggcggggacctgggcatcaggcatggcagaacccaggggcggccctgttgatggcagtcttcccttcttccttccaggtggcatttacaccctacgccccggagcccgggagcacatgccggctcagagaatactatgaccagacagctcagatgtgctgcagcaaatgctcgccgggtgagggcagccacgggggcactcggggcccatgccctggaggagcgtgtgtgtacaggggctggggcgcaagagcatagcccttgattcttactgaactcctagttctatgcactggcccatgctccctgctgcttctgggcctgtgaacatgctgttccctcttcctggcacacttcccaactccctttccctgattaactccaacttgccctttagacctcagctgaagatgtcccctcttccaggaaggctgcctgccccatactgcccagccggtggaggagggggaggaggagcctaaattagctcctgggggagtcagggagggctgcctggaggaggcagcactcagcttgaaagacaagtgctgcctcctttgagctctcactggcctctgatgttcccatggaagctctttccttgctgtgggattatagcccggtcctgcttcctgttgcctccactgtgtgctcctctagggcagagattgtggcttgttttctgctgaatccccagcacgtggcgcaatgccatgtaggtgctcagtgcatatttgactgactctgtgaatgcttacccatttcacagatggtagacctgaggcccagccacagttggtggagctaggtagcctgactcctggtgccctccatctattcatttgtgtctgtattcattcatgtcatgattataaggtatctgctgtgtgttctaagtgctgggaatacacagagagcagggcagacaaaacccttgccctcgtggagtctgcattttaacggtggatgcagacagatacattaggagatgtgtggtcctgtctatctgtaagtgctgtagaaagacaaggtcaggtaaggcgggggagacagaacgggacatactgttttacacagggtggtctgggaaggtctctctgaggaggtgacatttgggcagagccctgcaggaggtgagggagcaggtcatgcatgtatacagggaacagtgtgccaggaggaagcaacagcatgtgcgaaggccttgaagtcggagcctgtttggtgagttggaggaacagcagggccagcatgtgtggcccaggatgagcgaaggcgagtacggtaggggaggaggaggaaggagtgagcagggaccatggtaaggagtttagattttattctgtctgggagccaatggagggctttgagccgttaccttgagatgtaggtgggcatatgagtacctgtcaccgtccctagccattttaagacatcctagggaaagtgactctcttctttcttttattaactggaagggtctctttaagaagttactagagaggctgaggtgggcggaccaccggaggccaggagtttgagaccagcctggccaacatggtggaacccgtctctactaagaatacaaaaaaatagctgggcataatggcaggcacctgtaatcccagctacttgggaggctgaggcaggagaattgcttgagcctgagaggcagaggttgcagtgagccgagattgtgccactgcactctagcctgggccacagagtgagattctgtctcaaaaaaaaaaaaaaaaaaaaaagcagctactgagtcaacttttttttaaggtttccgttggtgttctctgtccctggaatgcctgctttccaggcccatgcccttgtccttgataggataccagggactacattcttactacctgttccccctatcattcatgcccctagctggagaatattagccatctatcaagaaggaagaaactggcaagctagttcttactaaagtgtgattgactgataatagggctccagtggtggaggttcaagcatctggaaagagcagagaggaatctatttttgagcagaaggggttcagaaatgacgtgatagctggtacaatactagatgggagatgattctgaggaattggaactccacagaatagccttcccagctgggctttagaactctggactttgtggggacagtggatgagcccagggtcctggcagaaggctcgcccagctgagacctctggcccttgtttcctcaggccaacatgcaaaagtcttctgtaccaagacctcggacaccgtgtgtgactcctgtgaggacagcacatacacccagctctggaactgggttcccgagtgcttgagctgtggctcccgctgtagctctggtgagtaggttcagagaaaaagggggcccttacacccctgcctccaacttcccccggcaactccagcctctttggcttccagctgtctggagttaccccaggctggttgttggaagtggcacaggtgcagctgtttacccctaccactggcattttcctcctctgtctcaccaaagcctcttcacagccccacggggcaggcggtgggagaactgtgcccacgtgagggttgaggaggtggtgcgtgggagagtggtgcgcatgctcgtgctgcgaggagcaggactgcggggaggagcgaaactgctgggaagagcgggactgcggggaagagcgggacttcggggaggagcggcactgcggggaggagcaggactgcagggaggagcgggactgtggggaggagcgggacttcggggaggagcgggactgcgggggacgagcgcgactgcgggggacgagcaggactgcggagagtagcgggactgcggagagtagcgggactgcggagagtagcaggactgccggtcctgcccctggactctggccggtgttgtgtgtgccccatgctgaggcggtccgccagcctcctggagatccgctgtctgagagtgctgggctgtctgggagggcagcgtgggtgtggcggaggcaggcgtgaccgtttgccgccctctcgctgctctagaccaggtggaaactcaagcctgcactcgggaacagaaccgcatctgcacctgcaggcccggctggtactgcgcgctgagcaagcaggaggggtgccggctgtgcgcgccgctgcgcaagtgccgcccgggcttcggcgtggccagaccaggtacggggtggggctcaggtccttggggacgcccatgggcctctcctttgtagacatccttgcagtgtcacgggcatcaacccattaattagtccagcagggagcactgttagtggtggccaggtgcctgctacccatccgtctgtccacctgtccaccgttcattcttcctgccagcactcccgattaggcacctcttatgtactggaaccaggagacccagagatggatcagaccaagccctaagctaggaaagttatgtgatgctgcaagatgaactcacataactctacagcccaatcccgtgcatgtgtgtacaggaatctgtgtgtgtgcatgtgtgtacaggcatctgtgtgtgtgtgtgtgtgtgtgtgtgtgtgtaaggggtggaggtgcagacagagctccttgggcccctcagacctctcctagggctctagtgccaaggcccagctgtcccgcagagtgtctgagtggttgacaagttcggattgttccctgaaggaactgaaacatcagacgtggtgtgcaagccctgtgccccggggacgttctccaacacgacttcatccacggatatttgcaggccccaccagatgtgagtagctgagtcctttggttctggaggagcagggaggggctgtccctgggtgactgtgggtccaggacacagagcagctcaccaaccaccattgtccagactgctttatctgagggtggctcccaggataaatggcatggtgggcaggaccttgccctggaaggcaggactgggtgggtgcatggggaggtgggggagggctaggagggggtggtcctcagagagggcacacatcgtcactctcctatcctgcctgctggggcccgtgaatgagcccagccaccccagccactctgtcccctgctgcctcctgaccaagcctcctcctcctccagctgtaacgtggtggccatccctgggaatgcaagcatggatgcagtctgcacgtccacgtcccccacccggagtatggccccaggggcagtacacttaccccagccagtgtccacacgatcccaacacacgcagccaactccagaacccagcactgctccaagcacctccttcctgctcccaatgggccccagccccccagctgaagggagcactggcgacttcgctcttccagttggtaagtcgcaagaagtctcattcattcactccttctgtctgcctgtctttctgtctctctttcttcctctcccatggttttactgagagcccacggggggctggaccctgtgccctgtcctgggatacaggtggcagtgagactgctttctccccacacctggtgctatcattcaaaatccctaagtgcgtgggctggatgcagtggctcaagcctgtaatcccagtgctttgggaggccaaggaggctggaggattgcttgaggctaagagtttgaggtcagtctgggtaacacagcgagactccatctctataaaaaaattaaaaaattatttgggtgggatggtgcctattgtcccagctactcaggaggctgaggtgggaggatcacatgagcccaggaatttgaggctgcattgagctctgatcgtgccactgcactccagcctgggcaatgagtgaggtcctatctcaaaaacaaaacaaaaccaaacaaaacccctggataggggagaggtggggtcagcaattcacctgaatatgcagatggtctccttgctgctgtttctgatgagcccattaggctaagaagacagcgggctgggccaggtcacctccaggggcttccattctggggtagaactgcatcaggccagaggtctcaaactagtggcccttaggctgaatgaggcacacagacatgattgctttgtaattggatttgagaatctccggcctagactcgcccctcatttgcaatgacccgaagcaccttgggtccctggcttgcctggctggcccctggtacatttgagtttgttttctgtagctgtctgagcttctcttttctttctaggactgattgtgggtgtgacagccttgggtctactaataataggagtggtgaactgtgtcatcatgacccaggtgaaaagtaagagtccatccttccttccttcatccacttgttcaggaagcttttgtggggtgcctcctgtgagtccagcactgggcacagccttaggggtcagacagagctggatatgggggtccttgttctgtaggagcttaaggcctggggtgaaggtacctctgctaacttaattactaaaaggcaagaggtgatcagggttttctaaagggtaggaggagttcaggattcctatccaggaagcctgggggattcgggcttcctgcagcaggtggtctctgagctgggtaagatcttgatgggtggagtctgtgcagggaaggacacgcatcctcagtggaggcgcggatggtatagatgggggactggagaatggttgggatggtggcaggtggagttgggtgggggcttctgtggaccttgtctggtaggcgattggtccccacagggctgggcctctctgctggttctatggggccccatactgccctcctacttaggacagatgtgcctgaggaagtcaatctcttacttgtcccctctcctctttatagagaagcccttgtgcctgcagagagaagccaaggtggtgagtgtctccactgccctctccccctcttcccctggtctccttcccggcgtgctgggctgtcacagaggaagcagtgaattctgtcattggtctgtccagtgtcaggaggtgtgcagagccctgggaggtggaggaaaggccggggagtcaggcagccctccatgggctaagagaggctgtgagtgtgaaatgctccggcagagagcagatgccttcgtggcgttcgtggcaggcacgtggtcgtggacccacagcgcaaccttgggcagatgtgaaattgctctatggctacttccttaccatgagatgggggttgtgtctgctcgatccagcctgcagggtggtgccattcggtcagctgacaatgatgtttctccttgcctccattgtgtttacagagcactttctcagagagcagtggttttcaaactgaattctgggatagcccagtgtcccacagagggcccttgggcgtgggggaagtggtcatctctcaggtttgaggtagaggctgtggggctgggccctgggtcctcccaaagcaactcacctttgatctgttttataaagtagggcctgcgaaggctttttgttagagacagaccaacagtgtgtcatatcatagtatttcattcattctccatcaggaaggcatttggctgcaagtaaccccaaacctacaggtgactttagaaaaaatggctttatttttcttgcattgtaagaagtcaaggggttggtgtctgctggaatggcctccactatccccttgcatggtgccagcaggaccccaggctctgtcatctttagtgtgttgacttttgttctcttgtttgtggcctcatgtcataagatggtaatcatcacttcatatgtcacctctaagtttgaggtgggaagaaggggcaggtggccaggtcagccatggtgcccttatcagtaaatcggatgccttcccagaagccctgggtagacttctttcatctcactgaccagacagtgtcacatgaccacccctagctgcgagggaagctgggaaagagggtgttttgcttttccagcctctatggaggaggaggacaagggaggggggttggaagtgggtatggggtgagccagaacatacgtctgtcacagccttgcacctggtaggcagggcaggttttttacccaatttgacagatgagaaaacagagtctgatgagttttctcgacctcaggggcaggtagagaaagaacttctcaacctcatggatatttgagacaacatcttacttaagggaggccaaggtgggaggattgcttgagtctaggagttcaagaccagcctgggaaacacagtgagaccctatccctaaacaaaattaaataaaataaatatttttaaaaaggatcttggctgggcacggtggctcactcctgtaatcccagcactttggaaggccgaggtagatggatcacttgaggtcaggagttcaagactagtctggccatcatggtaaaaccccatctctactaaaaacagaaaaattagccaggcgtggtggcacgtgcctgtagtctcagctactcgggaggctgaggcaggagagtcgcttgaacccgggcagtggaggttgcaatgagctgagatcacaccactgctctccagcctgggcaatagagcaagactccatctcaaaagaaaaaataaaataaaataaataaataaaatatcttacttagttgtgggggctgtcccgtgctattcagcagcatctttggtctttatttacttacatgccagcctcattcccactccagtggtgacaatcaaaaattctccagacatcaccaagtgtcccctggagggcaaaatcacccctagtggagaaccactgctcgagggaacagctcagccctgggcagcccaatacccgaagcttacaccaggtgtttggaatcagatagattgatttcatcccctgattttggtgacaagaaaagagatgcagggaggaaaactgagttgctcaaggtcgcaccgcagtgtgtctctggactcccatctcagtgctctttgccctgccctacagtatttcagtggggaggaaattttctcattccccggcgagcgagtttcactgctccctttctccagcttcaattcagtgacactgacggttgccgcctggtggcgtgcgtagagcaggtgtctcccccaagctcttccgcagcagcccagctgtcaccttccctttccccaccaagcgtttcccaatcctctgtgcactgaagatgtcctgggtgtggcctagcagcctctgcttcccttttccattttttttttctttctttctttttttttttttgagacagctatgtcgcccaggctgcagtgcagtggcgccctcttggctcactgcagcctccgcctcccgggttcgagtggtcatcccacctcagcctcccaagtagatgggactatgggcatgcgccaccatgcctggctaatttttatatttttagtagagacggggttttgccatgttggccaggctggtctcaaacccctgacctcaagtgatctgcccacctcggtctcccaaagtactgggatgagaggcataagccaccacgcctggcccctttcctttcactgttgctctcagtgttcactgaatgtgagtgactcaagtatctgttgagtgccccagtggtgtgtctagtgcagaaaaaaacccccaaaccctgatttgtggtgtttgctaatttctgtggtataaacactcacactgtagccagtttccaactcccaagaccttcctgaatatggagttgggaggaaatctgcacaggcctgagcttatcccagcacagccctggctgagccctgccaggctctttgtgactgagtccccacgcatccctgtggggcagggagcatcatcacccccattttacagaggaggaaactgagactctgggaggttccatttttcctgtaggattagatcattaggtgagtggcatagcccaggtttgaatcaggtttatgcctgtgtcccacgctactcctcaaccagcagctactcctgataagaggccagtggagagtcctcttgagctgggctgctgggcttagagtgtggactcagcacccacctgctcctcctgccacagaaagaacgtccagggcatgggagacagtggcgttcctttgtttagaaaacaccaacatgtggccgggcgccatggctcacgcctgtaatcccagcactttgggaggccgaggggggcggatcacgaggtcaggagatcgagaccatcctggctaacacagtgaaaccccatctctactaaaaataaaaaaaattagccgggcgtggtggcgggcgcccgtagtcccagctactccggaggctgaggcagaatagcgtgaacccgggaggtggagcttgcagtgtactgagatcgcaccactgcactccagcctgggcgatagagcgagactccatctcaaaaaaaaaaaaaaaaaaaaccaatatgtgagcttacccacaatcacccccatggacacggacacactcatgcacggacccacgtctgataacaggtgcgaacatttatcgggtgttgaacggatgccaggcactgtgcccagcgttctttattctcacagccatgctgccacacgcaggcagtatgattcttgtcccccattatatggcccaagaatcatgggcccagagaagttagtaactttcccagtgtggcacagctaatgatcacggcctgggacacgaacctaggagtgtctctcctcgccaccccagcgcacacactcactacgtcactcacagatatgcacacatgcccccaacatagacacacgtgtgcacgcttcacaccctcacgcctgtagacacaggtgtgtgagccttgtgaacacacaaacagacggacacagcaggaacctggaggacctggcccgtggctctgctgggtctctgcttctgcccagcagggctgggccaggaggggccgggagctgagggtgctggctggctggctggctggctggaattctgtttttttttttttttttgagaaagagtcttgctttgtcgcccaggctggagtgcagtggcacaatcttggctcactgcaagctccgcctcccgggttcacaccattctcctgcctcagcctcccaagtagctgggactacaggcacccaccagctcgcccagctaattttttgtatttttagtagagacggggtttcaccttgttagccaggatggtctcaatctcctgacctcgtgattcggtgaccacctcggcctcccaaagtgctgggattacaggtgtgagccactgcgcccggccctgggatcctgtgttttgaatgaggctcctcagtactcggctctactggggtcccagcccaaggaataggactcagcctgcttctgtgccacctggggctgcttgaactttgcgacttgtggcttgggaggagggaggtggccgtgacctttgggggtttttgttctgcctggctgtagccaccagcagagggggtggggcacaggccagaaaaaccccttttgtggggttgtgaggagtgacaattggctgcttctcctccccttccaggctcagagcagggctggggggcagttgtgggcagtgaccagggtcagaccacctgggcggaggttcagcatgaacttgcaatgccctccatctctccaaaactgggggacccagcccagggagggtgtgggggttcctggggaagctggtctaggcttctgctcctgccacggaccagctgtgtgatgctgggcacaggatgcactttctctgggcctccgtggcctcttggggatggcttgcacgagatccctccagtcctgagtgagaggctgtggccttggggaattaagggtgcaggtggcgctcaggtgtccgagaagccatgggagccgggggctgcagggattggacagagaggaccctggtactcgcatctgttctcagaccacatctggaattgtagctccctctggagggaggcaggaggtctcagcctttcttggggggcggtggcacctgcgctgctcgctccacccctgctctcacctcccgctgcagtgctggcgagccccatcagcccttcactcatctctaccctccttctttctgcctgggacacttgttttcatcctgggcaggccaggggccagggcagctgttgggaatgtggcctgtgccatctccttttttgctgggatcagaaaacaatcgcttagaattccaaggcaagggtgtgagcgcctggccagccagtgggaacagacaacagcctgggagaggaatttccagcctctcttcagtgtgcgtgtctggaaatggggaccttgccttgagcctccagagttgaaaccccagacacccaggaaaggccctttgggatttagcccagccacagtatgtcctaaccgtgaccttgggcaagtaactcaatctctccgtgcctcagtttccacaaagcaaggataacactgggttgttggaagaatcaatatagatattgtctggagggatgtaggtacagtgcatggcattgggtggcactcaaatgtcagctaataatattattattattctacgggaagaagacatcaggggaagttgcagagcagcctgtgggcggactctggaacaagaggctgaggcagtgcagcagagggtctcagacgtgagcgctctctgccccggaatgattgactgagcgcaaaggtctgcacgctttctctgtaaagggccagatggtaggaatttcaggctttgtggactgtatggtctcagtgacagctactcaaacctgcctctgtagcaagaaagcagctacatgcatagacagcacacacccaactgagagtggtgtgttcctatctaattgtgctactggacacccaaacttgagcttcccaccattccatgtgccgcaaattattctttttttttgagatggagtttcactcttgttgcccagcctggagtgcagtggctcgatctcgcctcaccacaacctctgcctcccaggttcaagcgattctcctgcctcagcctcctgagtagctgggattacaggcatgagccaccacgccagctaattttgtatttttagtagagacggggttttgccatgttggtcaggctggtccccaactcccttcctcaggtgatccgcctgcctcagcctcccaaagtgttgggattacaggcatgagccaccaagcctggccacaaattattcttaaacatttttttttcaaccatttaaaacatgaaaaccagtggggtgtggtggtgcacgcctggtatcccagcactttgggaggccagggtaggaggatggcttgagcccaggagtacaagaccagcctgggtaacatagcacaaccctgtctctacaaacaatcgacaacaaaaaaattagccaggagcagtgacacgtgcctgtggtctcagctactcaggaggttgaggcaggaggatcacttgagcctggaaaatcgagggctatagtcagctatgattgtgccactccactcctgcctgagcaacagggtgagaccctgtctcaaaaaaaaaaaaaaaaaaaaaaagtgaaaaccattcttagtggcaggctgtactgggcctctgggcaatcatttgcctagttctgatttaacaaactcttgtatggagtttactatgtaataggcattgttttaagcactttacaaatattcagccatctaatcttcacaacaaccctatgaggtaggctattattctccctttatagagtaaaaaaaaaaaaaaaggcacagagaggttaagtaacttgtccaaggtcacacagcaagtgagtggtagagtcatgatttgcacttgtgtggcctgggtttagagtccacactcttggttgctaggctgggccatgtctccctgtgcagatggggtgaaggaaagctgctttccttctactcccttatgcaaaataaggatgaaaatcctgccccacctctaagactatttggtgaacagggccaggtattctctgccctcataggacactctagtagagcagctgggtgctaataacagaaacacagaaaccacggagaatcacacctcccaaaaagtgccgtgtgtggaaagaacgtgcaagggtgggcagaaacgtcacgtaaactgagaagtgctgatggcaggaggtgtggatggcagtgggaaggaagaggggaagaaagagctggctggtgggctgactgctctcccctaccaccccctgcccatccagcctcacttgcctgccgataaggcccggggtacacagggccccgagcagcagcacctgctgatcacagcgccgagctccagcagcagctccctggagagctcggccagtgcgttggacagaagggcgcccactcggaaccagccacaggcaccaggcgtggaggccagtggggccggggaggcccgggccagcaccgggagctcaggtaagaggtgggagcacacctggcttcttcccaagcctccttggtctttctcacctggtttctgtcttagccatctcctcctgagcctccccgcagggtgggacgaggcctgagccacagggaacttccttcggttcgctgaacctaagttccctcccgcctttgcccatgctgggcctatcacctcaaaatcctcccttctgtgggacaaccccagcttgtccaagtccctggtatctgggggaggagttttcctgaaaccttctccctgctaccacccccagctggcctggctgctcctccgggctcaccatgccctggcctccctttcacaggactgtcagactgcatgtacagacattgtcttctcctgtctcccacgccaggctgtgggacacctggtgagcctggatcatctcattcatccctgtatctgcaggcccaacacggcccagctactgataattaatcataacaatcgcttctacttatggaaggctacggaacagcaggcactgtactgggcactttacatgcataaaactgacctgcatgtcaatgctaagagatagttcctgttgttatcccattttacagatgaggaaactgagccccagagaggttaaacagcttcttcaagggcacatggctagtaaacagaagagccagactcacccctaggctgtcgggctccagagccctgggattggaagatgaatgaagaaatggtggctccagggctccactcactgcagtttgttgctgggtctctttaggtctgaggcactgggactgtggggattgtgtcccatttatgcaggctgcattgtgccctggacctggtctatgacagatgtcactcctggttggcatctctagggcccacactggaggggcccctgtacagggtctgctggcctgtgcctctctccctcttacctggcagtgccagccagtgagaattcagggaatgaccatgaacttgggtcagtctgagatccttgcctggccactctggtgccataagaatttgggtgggatgcttaaccctgccaagccttggttttttcacctagaggtgagctatagcgcctccttgccagggctggtgagagatgggtgacattgtgcccagctgggcaccagaccagggccaggctccctctgggccgcctccaggtggggactgatggctgcagcccccaccacgcagccctcctccagctcactcacccccagctgctccccagctcactgcgcccctgcctcttgcctgcactcatgccacccctgcctgccacacctgttcctacctgcccccaactgcccacaggagctgacgtggccatttctgtctgccccatcatagcccccagcctcctcggtgggaggtctcatcagtgcccctcactccatcctgagaactccctatgggagggcctgggccagtgcctggaagagatcaggggccctacacactgttgaatgaatgaatgaatgagtgcgctccaattataaactcttagtctttgcccagttcttggattcgtctgattttttttttttaaatggggtctcgctcgtcgcctaggctggagtgcagtggcgcagtcttggctgacttatctgctcaccgcagcctccgcctcccaggttcaagtgatcctcccacctcagcttcccgagtaggcgggattacaggcatgtgccatcacgcctggctaacttttgtacttttagtagagatggagtttcaccatgttggccagactggtctcgaaatcctgacctcaggtgatccatctgcctcggcctcccgaagggctgggattacaggcgtgagccaacatgcgcagcccatctttctgatttcttagctacacctggtgtggctccctccttgggccagggtggagccctgaccatgtctgccctcccctctcccctctgccccttctgctctgtgctccttctcccgagtcccccagcccgtgtccctggcctctgtcttctctttctctccctcccacccctaacacctccctccactgtgggaacctgtaaaccccagggttgtgccccttcatggtcccccatccacccccgcaatgtctcatgctcgatatacaaaggccatggtgactttgggtgacatttgggtgctgtggaggctcagggtggaaatttccttccggccttgtgatttcaaccctcctcccccaccacatgcttggggctgttttgagcacagcaggttgccagctccatccacctcccggctaccctatccgagtagttggagttagggagaaccaggctggggtgagggcactcagcaggcccctgcagcaacagcagcagcaactctcattttctgagggggctacttactgtatgccagtcccttcatattcatctcagcaaacccaccgtccagtgcctccccaaccagttagaaaactcagttgcccacaggggctgggcaggaaggtgaggcaaaccttgggctgtccttggccggatctcctgcatctggctcccaagggaagccataaatccagatttttaaatgtaaacgcctgaattttaaatgttggtaatcaattcacttaaaaacatcaccaccaccaccaccaccaccaccaacaaaaaaacccgtagacttgtccctgttacaggcactaggaacacagcagggaacaatcaaaaagtccctggtctggccaggcaaggtggctcatgcctgtaatctcagtacttcaggaggccaaggcaggaggatcacttgagcccaggagttcgagactagcctgggcaacatagcaagacccccgtctctactaaaaaaataaaaaaaaaagtccctaccctcctgggttcagagtctggttggggaccccaggagctgggggctctggagatcaggagatcacagaaatggggagggacccagagagtggtggataggatgggaagtaaatgtctctagagagggaggccagggggtggagggcgcttcgtggaggaggtggcctttgagctaaggcctgagcactagagaagagctctctaggctgagggagcggcctgtgcaaaggcccaggggacctgaagggctcaaggggctgtagcagggggtggggaatgtggctggaaggaaccccatcaaggtcttggagcggcaggagagggggtgggagaaggcaggctccagatcagacagggcctggtaggctgtagcaaggactgtgggtttttgagcccccaaggaagtgatctgccaggttcaagggccagctctggctgctgatgggaaacagatttcagaggggtggggttgaagccaggacagatggaggctgttcacacccatccagatgggagtgaggggaggcttccatagcccaccatgcagcagcagggcagggtgacccttgcagaagtcatcttttgtttttgtttgtttttgagatggagtttggctctttcgcccaggctggagtgaagtgacgtgatttcggctcactgcaacctccgtagcctgggttcaagctattctcctgcctcagcctcccgagtagctgggattataggcacctgccaccatacccggctaatttttttttttgtattttgagtagagacagagtttcaccatgttggccaggctggtctcaaactcctgacctcaggcgatccacctgccttggcctcccaaagtgctgggattacaggcgtgagccaccctgcctggtccagaagtcatcttttgaagggagacaaggcaggaatgatggatgggtgtgtgatatgagagaaagatgggtccgaggctctgggcccaagcagctgggtggatggcagcaatgggaactgtgatgagcaggagaggttttggatgcgagatgggagtagaatcaagagttaagttggaggctgagcacggtggctcacacctgtaatctcagcgctttgcgaggctgaggtaggcagattctttgaggtcaggtgttcgagaccaacccaggcaacctggcgaaaccctgtctctacaaaaaattagcagggtgcggtggcctgtagtcccagctattcaggaggctgatgtgggaggatcacttgaggccgggaggcagaggtcacagtgagttgagggagtgacacagcactcttttgagaccctgtctcaaaaaaaaaaaaaaaaaagacagaagagacagggtctcactatgttgcccagtctggtcttgaactcctgggctcaagcgatcctacaaacttggcctcccaagtagacatctgttttatataattggctcctcccatctctggggtgattggggctgggtaggtagtgatgctattcttattcggcagaggggaaaatgaggcacatgcaggttaagtgacttgctcaaggtcacacagcagagctgggctagaatcttggtctcggctcctggcccagtgctctttcccatgtgtctgaatctgcatcttgggcaggggtccctgggccccactcctggacccccggactgacccccaccccatcttgtgcttagcagattcttcccctggtggccatgggacccaggtcaatgtcacctgcatcgtgaacgtctgtagcagctctgaccacagctcacagtgctcctcccaagccagctccacaatgggagacacagattccagcccctcggagtccccgaaggacgagcaggtccccttctccaaggaggaatgtgcctttcggtcacagctggagacgccagagaccctgctggggagcaccgaagagaagcccctgccccttggagtgcctgatgctgggatgaagcccagttaaccaggccggtgtgggctgtgtcgtagccaaggtgggctgagccctggcaggatgaccctgcgaaggggccctggtccttccaggcccccaccactaggactctgaggctctttctgggccaagttcctctagtgccctccacagccgcagcctccctctgacctgcaggccaagagcagaggcagcgagttgtggaaagcctctgctgccatggcgtgtccctctcggaaggctggctgggcatggacgttcggggcatgctggggcaagtccctgactctctgtgacctgccccgcccagctgcacctgccagcctggcttctggagcccttgggttttttgtttgtttgtttgtttgtttgtttgtttctccccctgggctctgccccagctctggcttccagaaaaccccagcatccttttctgcagaggggctttctggagaggagggatgctgcctgagtcacccatgaagacaggacagtgcttcagcctgaggctgagactgcgggatggtcctggggctctgtgcagggaggaggtggcagccctgtagggaacggggtccttcaagttagctcaggaggcttggaaagcatcacctcaggccaggtgcagtggctcacgcctatgatcccagcactttgggaggctgaggcgggtggatcacctgaggttaggagttcgagaccagcctggccaacatggtaaaaccccatctctactaaaaatacagaaattagccgggcgtggtggcgggcacctatagtcccagctactcagaagcctgaggctgggaaatcgtttgaacccgggaagcggaggttgcagggagccgagatcacgccactgcactccagcctgggcgacagagcgagagtctgtctcaaaagaaaaaaaaaagcaccgcctccaaatgccaacttgtccttttgtaccatggtgtgaaagtcagatgcccagagggcccaggcaggccaccatattcagtgctgtggcctgggcaagataacgcacttctaactagaaatctgccaattttttaaaaaagtaagtaccactcaggccaacaagccaacgacaaagccaaactctgccagccacatccaaccccccacctgccatttgcaccctccgccttcactccggtgtgcctgcagccccgcgcctccttccttgctgtcctaggccacaccatctcctttcagggaatttcaggaactagagatgactgagtcctcgtagccatctctctactcctacctcagcctagaccctcctcctcccccagaggggtgggttcctcttccccactccccaccttcaattcctgggccccaaacgggctgccctgccactttggtacatggccagtgtgatcccaagtgccagtcttgtgtctgcgtctgtgttgcgtgtcgtgggtgtgtgtagccaaggtcggtaagttgaatggcctgccttgaagccactgaagctgggattcctccccattagagtcagccttccccctcccagggccagggccctgcagaggggaaaccagtgtagccttgcccggattctgggaggaagcaggttgaggggctcctggaaaggctcagtctcaggagcatggggataaaggagaaggcatgaaattgtctagcagagcaggggcagggtgataaattgttgataaattccactggacttgagcttggcagctgaactattggagggtgggagagcccagccattaccatggagacaagaagggttttccaccctggaatcaagatgtcagactggctggctgcagtgacgtgcacctgtactcaggaggctgaggggaggatcactggagcccaggagtttgaggctgcagcgagctatgatcgcgccactacactccagcctgagcaacagagtgagaccctgtctcttaaagaaaaaaaaagtcagactgctgggactggccaggtttctgcccacattggacccacatgaggacatgatggagcgcacctgccccctggtggacagtcctgggagaacctcaggcttccttggcatcacagggcagagccgggaagcgatgaatttggagactctgtggggccttggttcccttgtgtgtgtgtgttgatcccaagacaatgaaagtttgcactgtatgctggacggcattcctgcttatcaataaacctgtttgtttta

SEQ ID NO: 13 - DNA, 3682 bp, Homo sapiens
  source 1..3682: mol_type = genomic DNA
gcgagcgcagcggagcctggagagaaggcgctgggctgcgagggcgcgagggcgcgagggcagggggcaaccggaccccgcccgcacccatggcgcccgtcgccgtctgggccgcgctggccgtcggactggagctctgggctgcggcgcacgccttgcccgcccaggtggcatttacaccctacgccccggagcccgggagcacatgccggctcagagaatactatgaccagacagctcagatgtgctgcagcaaatgctcgccgggccaacatgcaaaagtcttctgtaccaagacctcggacaccgtgtgtgactcctgtgaggacagcacatacacccagctctggaactgggttcccgagtgcttgagctgtggctcccgctgtagctctgaccaggtggaaactcaagcctgcactcgggaacagaaccgcatctgcacctgcaggcccggctggtactgcgcgctgagcaagcaggaggggtgccggctgtgcgcgccgctgcgcaagtgccgcccgggcttcggcgtggccagaccaggaactgaaacatcagacgtggtgtgcaagccctgtgccccggggacgttctccaacacgacttcatccacggatatttgcaggccccaccagatctgtaacgtggtggccatccctgggaatgcaagcatggatgcagtctgcacgtccacgtcccccacccggagtatggccccaggggcagtacacttaccccagccagtgtccacacgatcccaacacacgcagccaactccagaacccagcactgctccaagcacctccttcctgctcccaatgggccccagccccccagctgaagggagcactggcgacttcgctcttccagttggactgattgtgggtgtgacagccttgggtctactaataataggagtggtgaactgtgtcatcatgacccaggtgaaaaagaagcccttgtgcctgcagagagaagccaaggtgcctcacttgcctgccgataaggcccggggtacacagggccccgagcagcagcacctgctgatcacagcgccgagctccagcagcagctccctggagagctcggccagtgcgttggacagaagggcgcccactcggaaccagccacaggcaccaggcgtggaggccagtggggccggggaggcccgggccagcaccgggagctcagattcttcccctggtggccatgggacccaggtcaatgtcacctgcatcgtgaacgtctgtagcagctctgaccacagctcacagtgctcctcccaagccagctccacaatgggagacacagattccagcccctcggagtccccgaaggacgagcaggtccccttctccaaggaggaatgtgcctttcggtcacagctggagacgccagagaccctgctggggagcaccgaagagaagcccctgccccttggagtgcctgatgctgggatgaagcccagttaaccaggccggtgtgggctgtgtcgtagccaaggtgggctgagccctggcaggatgaccctgcgaaggggccctggtccttccaggcccccaccactaggactctgaggctctttctgggccaagttcctctagtgccctccacagccgcagcctccctctgacctgcaggccaagagcagaggcagcgagttgtggaaagcctctgctgccatggcgtgtccctctcggaaggctggctgggcatggacgttcggggcatgctggggcaagtccctgactctctgtgacctgccccgcccagctgcacctgccagcctggcttctggagcccttgggttttttgtttgtttgtttgtttgtttgtttgtttctccccctgggctctgccccagctctggcttccagaaaaccccagcatccttttctgcagaggggctttctggagaggagggatgctgcctgagtcacccatgaagacaggacagtgcttcagcctgaggctgagactgcgggatggtcctggggctctgtgcagggaggaggtggcagccctgtagggaacggggtccttcaagttagctcaggaggcttggaaagcatcacctcaggccaggtgcagtggctcacgcctatgatcccagcactttgggaggctgaggcgggtggatcacctgaggttaggagttcgagaccagcctggccaacatggtaaaaccccatctctactaaaaatacagaaattagccgggcgtggtggcgggcacctatagtcccagctactcagaagcctgaggctgggaaatcgtttgaacccgggaagcggaggttgcagggagccgagatcacgccactgcactccagcctgggcgacagagcgagagtctgtctcaaaagaaaaaaaaaagcaccgcctccaaatgccaacttgtccttttgtaccatggtgtgaaagtcagatgcccagagggcccaggcaggccaccatattcagtgctgtggcctgggcaagataacgcacttctaactagaaatctgccaattttttaaaaaagtaagtaccactcaggccaacaagccaacgacaaagccaaactctgccagccacatccaaccccccacctgccatttgcaccctccgccttcactccggtgtgcctgcagccccgcgcctccttccttgctgtcctaggccacaccatctcctttcagggaatttcaggaactagagatgactgagtcctcgtagccatctctctactcctacctcagcctagaccctcctcctcccccagaggggtgggttcctcttccccactccccaccttcaattcctgggccccaaacgggctgccctgccactttggtacatggccagtgtgatcccaagtgccagtcttgtgtctgcgtctgtgttgcgtgtcgtgggtgtgtgtagccaaggtcggtaagttgaatggcctgccttgaagccactgaagctgggattcctccccattagagtcagccttccccctcccagggccagggccctgcagaggggaaaccagtgtagccttgcccggattctgggaggaagcaggttgaggggctcctggaaaggctcagtctcaggagcatggggataaaggagaaggcatgaaattgtctagcagagcaggggcagggtgataaattgttgataaattccactggacttgagcttggcagctgaactattggagggtgggagagcccagccattaccatggagacaagaagggttttccaccctggaatcaagatgtcagactggctggctgcagtgacgtgcacctgtactcaggaggctgaggggaggatcactggagcccaggagtttgaggctgcagcgagctatgatcgcgccactacactccagcctgagcaacagagtgagaccctgtctcttaaagaaaaaaaaagtcagactgctgggactggccaggtttctgcccacattggacccacatgaggacatgatggagcgcacctgccccctggtggacagtcctgggagaacctcaggcttccttggcatcacagggcagagccgggaagcgatgaatttggagactctgtggggccttggttcccttgtgtgtgtgtgttgatcccaagacaatgaaagtttgcactgtatgctggacggcattcctgcttatcaataaacctgtttgttttaaaaaaaa

SEQ ID NO: 14 - protein, 461 aa, Homo sapiens
MAPVAVWAALAVGLELWAAAHALPAQVAFTPYAPEPGSTCRLREYYDQTAQMCCSKCSPGQHAKVFCTKTSDTVCDSCEDSTYTQLWNWVPECLSCGSRCSSDQVETQACTREQNRICTCRPGWYCALSKQEGCRLCAPLRKCRPGFGVARPGTETSDVVCKPCAPGTFSNTTSSTDICRPHQICNVVAIPGNASMDAVCTSTSPTRSMAPGAVHLPQPVSTRSQHTQPTPEPSTAPSTSFLLPMGPSPPAEGSTGDFALPVGLIVGVTALGLLIIGVVNCVIMTQVKKKPLCLQREAKVPHLPADKARGTQGPEQQHLLITAPSSSSSSLESSASALDRRAPTRNQPQAPGVEASGAGEARASTGSSDSSPGGHGTQVNVTCIVNVCSSSDHSSQCSSQASSTMGDTDSSPSESPKDEQVPFSKEECAFRSQLETPETLLGSTEEKPLPLGVPDAGMKPS

SEQ ID NO: 15 - DNA, 34503 bp, Mus musculus
  source 1..34503: mol_type = genomic DNA
agtcaccagctagagcgcagctgaggcactagagctccaggcacaagggcgggagccaccgctgcccctatggcgcccgccgccctctgggtcgcgctggtcttcgaactgcagctgtgggccaccgggcacacagtgcccgcccaggtgggtgactcttggggtcacgggggacagctgcgcatcacaaagtgcccattccagctactgctactgcacaattccgggacagcatgagaggccatcacgtccccagcagacacgcgccacgcgcctctggggacccactggggacccgaggtctggcccgttgggatcctggggtggtactcggttcccgacagccttatgttccagaaatacccagtggctttctccgcgagcttgatcagggctcgaataacacccagcagggctcaggaacactgttcatccttgcgaaatcccttctgtcccgcggtctcgaggcgggaaggaccagggccactgccccattgcttgagcgggttgtgtcgtctgaagacttccttctctgcgccatggtctgtctctttcttagaaaccctgggattactagatgttggcggggccaggagtctaagtaagcgcctagtataagagaccgatggggagtgagtcacttctctgtcactagattgcttccatggatccgccttgctgtgttcaggggacgtttcagaatgttctcagtgtagtggcagagagggcagctaccccaaggaacctcgggaaaatggaccgattaaagatcccagtatccggtattcacattgcccccctcccccccccttcctgcctccattgatcgaagacagggtaaaaaaaggcagattacaggtacggaaaaatgaggaggctcagagaaattaccttttttgaaggatttaaagggagcttgctgcactgacatgcctttgcttggttccatgtatgctctctgcctcctgagcccaccttgatggacagggtgtgcttacctgactgcaggggagtagagtggaaggtggcttctgttgcgtccggaggtgatattcaatggtcctgggatgcaaaggaatggactcatccttggtgggtgtaggtcctcagggaggtgtcaaggatggactctgggtcaggacagtcccagttctgagggcggagtgtgaatgtgcatggttgtggtcaggagcctgagtggggattgtgctctgagctccaaggaaggataggtctttgggcactgagctggggtctgtccctggggacagacagagcacaggagcttctgtaccggatgggacacgcaaggctttgtgggatccacagtggtttggctgaaggtgtttccctcagacttccttccatacctgaccagtcccaggtcagcttagaccttctactactgttgcgtggactcttagctagtctgcctgtgttctaactcccacaaatcctcctttgacagagagaccttgctcaagcccagacacctctatctgggaagcctttgtagctcctagtggtggaggcagaacccttccttaccttcaaggtattccaggccagatggacatatctgtgttgcctgctcacatgaacctatgctctgtgaagctgatgactaggtgtctaccactgtgcgtgtatgacccctgcacacacattgtccatattacagatctctcaacacttctgagtcttttgtaaatgccaggtcaccagaaaggcctgtacacatccccccacctagacatgacctgctctatagagcacagattccatgctactttttattctctgtccctcaagggtagaagggacccttaacacagaactgtgcaagccttctcttgattgattccaaagaagctcctggtttgggacactcaagtgccagatactgtgttgggcactttgtcacagattagcactgaaacttcccttccagctgtttctacaaggtgggtaccgttgttccactgaaaggtgtggggatgggtgacaagctgtggcgtatgccaggaccacagaactgggaggtgatggggtgagatttgaaggcaagttgctagcctgactcccaacattctttctccagacattctcttacctgtattcccacttctatccctattgtgggactcagagatattgtgtgtagtgggtctgggcagcagagagagccctgaggatatttgagtaggttccaggggcagcaaacttactttacccttctattcagtctttcatttatttggcagataaataggtgtgaaacagggtaggtgagcacttgttctggtcttacttaacctgatatgtatggcctccctgtccctgggactctcaggactgaggactgctgtttgctgctcgagccagagtctgtagcatcccaggctgaccctggagtggattaggtacctgcagtactgctgaacctgagagctctttacttctttcctcctatctctgtcttgtgttcgttggctggcatccttctggggcatctgtattgtgactgaggatgtggcttggtattgggacctttagatggcggtggttaggtggtcaggtaccctgatatagagccatccatccatcaactctcttggcatttgtccatgcatgcttcacacactgcccactggacagctctaggaaactacctccagaaccccagaagccacatggccagaaggtcacacacttcagagacttgggttttgctcagaactgctcttgttacagttacatgggatacattcgcttttgtcgtggtaatagagaatttgcctggctttttttttttaatgatgatggtgtctcctgtagcccaggctggccttcaggtcactatgttgtttaggatgaccttgaagtccagatcttttttgcacatctccagagctaggattacagctgtgtgccatcaacacctgacgtatgtagctctggacttgtgtctctgcatgctgggcagcgctttaccagctgggctacatcctgaggccttctctggcatgcttgggttgaagaaagtcctggtccctggcccagtggcttcctgaaacatttgtccatctctaaggttgagtgacactttgacatgttttggcctttgctacccaatactagccagcgtagctttgtagggaaagagaagagttcacccagggtgtctttgtggggaagaagagagatgtttgccaccatgcctggtatatatatatatacatttcttgttgctcttgctgacagcttaatcacaacactcagggtggtacaggcaggattatcaattcaaggccatccttcggtacatgaagggtttgagataaccctggacttcatgaaaccaactaaaagaaaacaaaaaaactgaaaacatttgctaaatgtcagagatatttggctgacctttgttgtgactcgtgactccgttttacagccaaatgtgtcaggttggtgggcagatcggggttctggtggcccgcctctttcaaagtgtgtctgggcttgttcccactgctgtatcagatctgatgagctggagaccctctcctgaaagagctcacacttcctacctctactcatcctgggttatgatgatgccatcccagtggtggtggctcagggccttggagtgggcaaggagggaagttgagggttggcactgggagcagaagtgaggtgcatatgctatacccccaatttcagacaacatgagacaccagctcccttggtcagggcccaaggcctgatcacacagatgtcagccttcagccttcctctgttgtgatcagagcctccctcattcctttgtacagtggaaacacacccatggtgatggcaaggactaaggctttgaagtcactggtgtctgtcctgatttggttatattcagtgttcacagctaggaggaactcaggcacccatcagtgggagccataggtccccaaagcttaggcagcagatattcaattgccccaagttcctgtttgagtgaatttgctgcctggtacccccaaaccaacgttcttcctgtcaccttttcctgctgtacttcctgccccatatcccctggctgggcccctcagatcacttgtctgacttgggtctgggaccctgtgtaggaagcaaaagctatatggtcagggagtcaccatcttactctttcagtggccggtgctaaatgtcacttggggatgatgaggaatatgcatgatgaagttgaaaggagcacagaaggctctagctctgtgcttgtcaatttctaaatcatggccccttaggcatcatgggggggtcacctaagaccatcttgtatatcagatatttacattatgatttataacagtagcaaaattacagttataaagtggcaaaaaatataactttatggtttggggtcaccacaacatgaggaatggtattaaagggtcacagcattaagaagattgagaacccctattctagctcatccctacatgccaggaggtctctctcttaaatctcttccatctgcatttgtgtatatttatgagtgtgagagagagagagacacagagatggagagacagagagagacagagaaagatcttgcttacttaagacccaagatgggaaagccatcttctgaactgaagctgtctaattccctatgcccaagtgacttctaagacagtacaacctgggccagacggtggtggcgcacgcctttgatcccagcacttgggagggagaggcagatggatctctgagttcgaggccagcctggtctacagagtgagttccaggacagccagggctatacagagaagctctgtctcggaaaaaaaaaaaacaaaaacaaaaacaaacaaacaaaaacaaaaacaaaaaaagacagtacaaccttgaggaggaatcacagcctgagtgttagtagaacagagtttaatggcttgctgtgtgtcctttccatttatttaatctctctgagcctaagtcttccagcaacactaatctcaatgttctcccagaaggagtggagctggcagctacatgagccatgagaaaaaaagagctgatgtctttaccccttccttccttccttcctccctccctccctccctccctccctccctccctccctccctccctccctcccttccttccttccttccttccttcctttttgtatgtatgagcagtgtgcctccacatgggtagggatgtttgtctgtatgtaggtgcatgtctctgtctgaattgatattagatgtcttccttgaccactctacagtttacttgattgaggtgagtctctcactgagcttggagttggtctagctagccagcttgttctgggatctctgtttctacaccctaccccagcccctgtgctgggtttatagttagctgcctcatttatgtgggctctggagggtcctagctgtggtccttaggcttgtaggcaagtgttgttccccggagccatctctccagtccttcttgatcattttattcccatttcttttggttagaattatttccctgtcttaggcccccttggcaagatttaatggctgcccctcaggttgctcgaagctggggtgctgctgtctcaggcaggcctggaagtcttgggtttcctgctcctgtcccctagtgcctttgatatgtcaacagtgaggcatgcccccagatgctgaggaagtcagacttgcgtaacagccagcatgaccagctagtagcctccacgctcaagtaagcccaagtgggaagggtgtttcctcaaagaagctttttgtcactcattagaggggacgccttatttggtactgattctggcctgacagtatgtctctttgtcctaggatgcagggcaggggctttggggtttgggacccacctcttatgtaggacaggggctctgcagctctgggacctaccactctgatacctacacacatctttttccaccacggtactttgtgatgtcatagctgacagtgacaccattgtggtttggactgcttggctgtgagcaagagaagaggaagcaggcttagcttaccagcaggaggttgaggaagagagtgtccttgcacccccagtgtgagccatgctagggctcaggtgtgaaggtagctggtgtgttccaacctgtagctctgtctgacccttgccagcttgaataggatgatggaagactgactgacatcttgaaggtcatccacacccatcctgtttcttttgggttttttgtgtgtgtgtgtgtgtgtgtgtgtgtgtgtgtgtgtgtgtgtgtgtgtgtgtgtgtgtgatgttttgttctattgaaacagggtcttgctttgtagcttttggtcagcctggaacttgctttgtacaccaggctggccttgaactcatagagatccacaaatctctggttccccagtgctgggattaaaggtttatgccactacaccaggctccatttcttctttatggaggtggaggggttaggtttgtggatgctatgttgttcctcatttaagaaggcctgcacccagcccacccgttcagtgtgggaggctgcaagaggtcacacagtctgagtaggtgtgctctcctgtttaaactggaaagtgacagcatccagtgacctgctcaggggtgctgggtccttgagaggtcttgggaaccatactgttctctttgggagcctgggcctggggtgacccagcccctctgtcaagacacgaggaagacttcccactcaccaccactcaaggtgtttgtcagggaggccagtgcaggttgtctggttttgatcttgggccatagcaacctggagttcagaaaactgagtcagtctgaagttgaaaaccgagtgagaagagacttgcgggtagtcttgcaggccatgtacaaagacatctttttttgtcctctggggacagggcagaggctgtagatcctgagttctgacgtctggtatgacttccactttgggctggaccaagttgggcctccagttcccttgcctgttctgaatctccattgctccaagtctgacttctcaaagccagcattggaatccaggcctgcagctgttggacagtgggtgggaagctcagtagcttggagcagaggatggcgtgtaactggactggacagtggatctctgaggaagggctctggaatgttgactcgagtttcaggacccctgccaatgccctagctatgccctgtgcctggcctcccactgctgaccgacagcccagcttctggctactgctcacagagccaaggttcttaatgaggctgtgaccagctgcttgctctctggctgcctatgcctctggccatgagcctgggtcctgctgcttcctgctttctctggcaggagtccagccctctccagtcttagcccctcaggcctccactcttgcctctcggtggcttggtcctgtggtcacatcctcaccttgtctagtcacccatatgattctccctgaattctgccctcctgcaagagttcacagggaacttttctggccttgagtcccatagcatggcagactagaaatgagtggatgccaggtagaggctggagggactgggagcaggctagacccagtatctgggcaggaagtgtgctagaatcaacaaagactcatgaggctgtgtatctgcagccagtttgtgaaagaagtaatagcaactgcattaaacaattattggggccagttgtggtggattgaacaggcaatcccttgggtggtggaagcaggaagatggagagagttccaggccagcactgtctcaaaaagaaaatgtagtttgcaaaacaccttattgtgtgttatgttatgtaatttttttttaccagacccagacagtatgttgtcagattcattctatggagaaaagggttgggggaggaataatctttttttttatttgaaaatacagtgaacagggctggtgctggggcaatggttcaggagttagggacagaaactgctcttacagaggaccttggtttaatgcccaccactgaaacagcggttcattaccatctggaactgatatcctggggcaccagccgcacacacgtacatttaagaaaaacactcatacacataaaattaaaaataatagcaacaacaatagatgggctagggaggtcaggatcacttgctgctcttgcagaatccggggttctactcccaacacctacatggcaattaaatgtctgtaactccagttccaggggatcggttgcccattctggcctcttcaggcaccaggcacatacatcgcgcatagacaaacatgtagacaaagcattcatacaggtaaaaatgaatttatcttttaaaatgtaacaatgtaactaacaatgtaaatgtaaaaatgtaacaaatataaaagcaaaaatgcaacaaacaggctggggatacaattgtgcaagaaagaatttattacattgtgtaataaattaataatccaactgattaattaaaaaataaagctccaaagaaaaataattccttcaagatgcctgctaattagggatttaggctgagttcaaagccatacttccatacttttgtctgttgtcaactaacacactcttgccataagaagatgaggcgacaaggagccatccatagtttggaggcaaggagggagcctggggcagagagtaggtggactgatcatctggcctttgtgtggaggttcagaaagtctagagtcagggaggctcactgggaggctgcagtggtgactcaggtgaagtagggaggacagcagaggagggacggagagggggaggaccaagcgatgagaaagctggaggtaaggcatattttcccgtgtccccatcttccatagaggtttactgctcatcctgagctggttgacttgttttggtcattaaattgcctgaccttgaaactgctatgtatccgagggtgaacttctgatcctcctggttctctgcctcagttgctggaattacagatatgcaccaccatactgtctgtttgtttgtttgggttttttgtttgtttttgtttgtttttgtttgtttgttttaatgcagcgctaggcatggaaccaggcccttcaggtgtgttagacatcctctctaccaactaatcttcattctagccttctctgggtcacagtcagccacaggatcagccttgccataatcaccctggtcgcctactctgactggagtggatttgaaactgagctgaggtctgtaatgtctcctgagagccaggcatgtgccatgattaacccagcaggtgaatgagaagaaccggatgctgcacatggcttcggcaggtgtctaacaaatagtttcagtgataatcaacaaaagcaaaaggtctaatttcagagtgggtctgatgcactgaatgtaagaagcccttccattttcagccagtggggcagcaggccaatactcttgccagaggagatgagagggtcaggccttcttgtgcatggtactactgttcaccccaaccaaagcccagcttccatccataggctgcagaggctaccacccagatgtgatggtggttggttgtggccactacctgggctgtgatctgaaggctgcccttcagtttctggggatattgccttggccatttcttgaccagttctcatgtgagccaaacacagctcagtgaataggaaattagaactttcacttttgttgattagcgttgcatctatttattagacacctaccccagccatgtgcagcacccagttcttctcattcacctgcttggttaatcatgacactatgtatggtgggcatggctccgtttccattttgtagatgccaaaaccaagatggaagaataagagaaggaaagtcaaaccaggttctggctcaaagggagatcacagtagggtgtcagggaacacacaagttgaacagagttaactcaaatatgctctaacctgggaaatatacaaacagtcctaggttgtcagaggagccttctggagggatgacttccatctggggttcaggggtttatatgagaaagaggtgatggtgggatgagtctgaagaagctggggggtctgctctgcagaatacgtggtcagaggtagcagcaggagtcagggtgcagaagaggagtacgggagtcgtgtgctttgcgtcaggtggcagatgaaagctggcagcagaagctggagaagtttcattccagcctgaggacagctgaataaggagggccagtcctggaagtaggaagatggcttaggtctgtctgcaaagggaaatatgctagacaccaacagtgaggaaactagctggcaggagttgtccaggtattaaggagagccagttggagatgaagaaacccatatcaaagggcctcagggtaatagcagagagggtgaggcattctctgtcgttgaactgagtattatttgggggcagagcccttggcatgtagcctggagcctagccctaagaacaggatcccagcgtgggtttcctgtctgctgcagctcacttctaaagcacatcacaggcagcagtttgaaggagggatgtctcacccctgggccatctacctgtgatgtggttggtccttcctgacgccaatgctctttgtttccatgatggttggcaggcctggtcgcctaggccttgcgtcgctatgacagcctagcttgatgtggctgtaccgccatagtccatgggctcctataaacctccaagatcaagacttaaatgcaccccccccacaccttccatgcaaatgatgtggtctctctagtgcttgaagatagagcttccggctgagtggagggtccttgggcagacacctctgtctcatttgacctgggatgtggtggcccttttgcctggaaacatcatcaaactcttcaccactctgtaaagccagacaaaaatcatagggcatgaaatatctcagtcagtaaagtagaccagcacacgcttgggatcacagcactggggaagtggacaggcagatccccgggttcactcagtggccagtctagacaaattagtgaggcccgggccagtgagagaccttgtattgaaaccgagatggacaatgcactaagaagagctgacatctgacgtgcacatgcgcactcgcaagcacacacacacacacacacacacacacacacacacacacacacacacacacacttgtacccccatatgcacacacaggacagctgtgtgttcttgcacatacttatacatgtgtacctgcatacacacagaaaggtacacatgttcatgtgcacctgaacacacacaaacagttgtgcacacacacctctactcagacacacaaagaacacaagttataaaactgactgatgtagctgtgatgagttcccagtctgcacctacactgtatctcctggatctttcacttctacagtgatggtgaaatggactctgtcttagttactttttgatttctgtgaagagacaccatgactaagacaattcataaaagaaagcatttgactgggggctagcttacagtttcagagggtgagtccatggctgtcgtggcagggagcatgacaggcaggcaggtagacatggcgcttgaacaatagctgagaacttacatctgattctcaagcaggaggttgaggaagggagaatgggaaggagggagacacctcctggcatgggcttttgaaaccttgaaacccaccccccatgtcacacctccttcaacaaggccacacctccaaatccttcccagacaagagacaaaacttttgaatgtataagtttatggaagctattcttatccaagccaccgaaggcttgtactgacttcatttgtttggttcagagaaaaaggtggggaaatatatacaaatgctccagaatggcacttcacacagtaggtactttttctggatataagccttactagtctttctagcttatataaatggtgattctagtgggtatatactctttaccacaagctgggagttcttccaatgccaccttccctatcttgctctatacctgcctcagtgatagatctatacctagggtctattattctttcacctctcagtctgtccatctctacatccatctatctttccatctatctatttacccatccatctacccactcatcatttcatccatccatccatccatccatccatacatccatccatccatacatccatccatacatacatacatacatcctttctcccatctctccatccattcattcctctttccatttctctttccctccctctatttctgcatccatccatctccatctctccctccctccaatttttcatccatccacttctccatctatcctcttttcagtctttgcctaccaggtacagtaggtggttcattcttaccataggtttccagttctgacctggagccttgtttgctttttgttgttttgcttgtatgtttgtttgtttctttgtttctagacagagtttctctatgtagccctggctgtcctagaactctctatgtagaccagattagccttgaacccacggagaacctcaggcctccaccaacttagctctgggattaaaggcatatgccactccactactccctgctggaggctttatcttctgagcaactggctcacacaaacatgctgacagcatcaagtgaagttggattcatttcctcatttctcagtgtctgatctccatgcactgggggtgggggtgaatctgtgtctctctaatttaaagtaaaagactagtcctccccagccttgggaatctccggacttgtgaaccctctctagtgcccccattcccacccccatccctctgcagtccctgtagtggccctgaggcccagcccccaagactatgttttggggctttgggtacctccctttgcaggagtgaccttttgttctgcattacgcaggggctttctgttcctcattgtttagtcctgacagagattgtggtttttttttctttcttctgtccaagggaataaacaggcctggaggttgttgagggaggcatgggcccctttgccagctgctgggactgggattacacatagcagcaggagaaaggaccagaaagtttattcttagtgaagctggggacaaggaggcccccttgatgatgggtggatcagtgagacagtccaacttggctgagtcaaggccctttcccatcaggccctcttcgtctggaaggaagttgtttctagccaaaacagtgtttctctgggccactagaagctgcccaggccacagctcagttaccaccacccaagggatatacctaccccagggctggcagggcaagtgttcccatgagatgcacacaccgacagcccgtgtgtggagccggaggctgctgtttgaggaagtagaggagggtgaagagaaggttcttagttaatgagacaaatagtttccccaggaaggctagtctgggagttttattggggacactcaggccttctgtgtcagttagcattctttggagtgatggatacaaatgagctatgacactgatttctggggtccaaggctcccctaattctgctgtgtaccttcctcactcctttctcccaacttaccttactttctccatgggataggatactcagaccacattgagtagagcagaggagtctctaatccccaggaagagttctttcttattttatctttcctctttatgagcagtgtggctccccagcccagagactctccccccttagatgtgaaagggtcagccagccattgatgtaccctttgatgtgtttgttacattagcagttctcatctgaacacaacacactgggtccgagcggttccacgtgtgagatgtttattgggaggggggcgcaggggagaaggtgacagcagaaagagaaggggaaaaagagagagagggcctccttagaagtgggaacaaaacacccttggaaggagttacagagacaaagtttggagctgagattaaagggtggaccatgtagagactgccttatccagggatccaccccataatcagcatccaaacgctgacaccattgcatacactagcaagattttatcgaaaggacccagatgtagctgtctcttgtgagactatgccggggcctagcaaacacagaagtggatgcccacagtcagctaatggatggatcacagggctcccaatggaggagctagagaaagtacccaaggagctaaagggatctgcaaccctataggtggatcaacattatgaactaaccagtaccccggagctcttgactctagctgcacatgtatcaaaagatggcctagtcggccatcactggaaagagaggcccattggacacacaaactttatatgccccagaacaggggaatgccagggccaaaaagggggagtgggcaggtaggggagtgggggtgggtgggtatgggggacttttggtatagcattggaaatgtaaatgaactaaatacctaataaaaaatggaaaaaaaaaaaggaaaaaaaaagagatattaaggaaaagtaaaaaaaaaaaaagagagagagagagggagggctgttccccttatttatatgaaaaaaatgacgtaacacaggtaaaggtgggaggtgagccaagtggattctgggaatatgctgcaggtcgcgctgtcacctatgtgatgtcataggtttgggaggtcctgatgcaaagacccttgaccttgagaacagtcagtgaggtcccagacagtgtggaacacccttatttgtgtgctcagactcaactggttgttttgtcaagaaatggaacggggaagtgccaggatattgtgtgtaggcatgtgcgcatgcgcttggatgtgtgtgcagctgtccagagggagctgcagtggctttttcagactgggtactcagcatggttctgcgacttccctcacccagctgtctgcatgaccttcctgaaaaggattgccttgatggaggaactcagagataggccagggcagcagatgcatctatgttcaagcttcttggccctggtgcccagggggaggctctcgcctcaaggaaatgacattagaattattaccttactcagggtagcaactattgattactcttttctgtctggctctggatagggtagctcgcactgcagcctccaatgggccctcatctggggttactgggtgagcatgaagacaaggcagggggctggctgtattgggttgcttatccagggcacggtgtgcacagtcgcctgaagagggaagcactctgtgtggacttttggccaaaggcgcaagaggcagctagggtactgtggcaggtccagaagagccaaagactgtccacagcatagaaccccagtcccttgagtcatggcttctggtggctttcagctgttatcactgagtggctgagcaaagagaaacatgataggctcagaggtcactcagtgcacagcactaggcaaggtagggtgatgctctccagacacagctggggatgggaaggggaaagacagaaagcagagccactgcccacagatcatgggagtttgtgcagtctatacagaccaaatgagcctaatagtaaggtcggcatcttctctgattggcttgtttgcagtggcttttcagagactgatccatgcctttgctgtgctaattgttggatattttatgtatctctcttgctcccatagaattgagtcaggaaccgatgtccagagagatagggacacttgattgactatgaccatacagcttctggatggaagaataagaaaagaagaccacatctctctaactctccacctttatctgaggagtcaggggattcatttgggttactggtttaataaacatttattaagctcctgctgaccatatgacggcagctgctggtacaatcaagagtgcggagcagccttcctctttaacctagaaccaccccttggtcatttccaggtgacatcagcagaggctgcaagggtgttgagtgtgtgttcacaccctctttgctcttgtagatccactcccatgtttgctcatgagttcacatttgtgcagaaatggctaattcatgcttgtccctaaagtttccaattgctgttccaccttctggaagaaaggctggggcttaggcaggtctctgaggtactgggatagacccagtggtgacagttgctgctgctgtacacttctgagaactgaggacctcttggagatctgagggagggctctgtgtttctcacagttggttctgtgccatgttgggtgtttttttgttttttgttttttctcctccccatttgtctccctttcataattatttatttaattaaaaaatgtgagtactcctgagtatatgtatgtgaaccacacacattcaggagtatgcagaacttagaagggagcgtcaggttacctggaactggagtgacagacagttgtgagctgccatgttggtgctgggaactgatcccaagttgtctccaagaatagtaagtgcccctaaccactgcgctatctctggagctcctcctccccatcctccccatcgctccctgctttcctggtctctccctggaagtgcttagcccagtcattgaaatcatggcctagagagacagacaggacccaggctcaaatctctgtcactgccttaggtgggtaacctgtgctcgttatgcctgtttcctttctatacaatggtcggagtccaacatggctggttgttagagaactgaatgcaataatacatccatctcaggtccaggctctggaagcacagcctgaggcatggcttcttgtaacaggagaaggctctcaggcaagagggtggggtggcaggatgtggcagcagggtcacatgttttccagccaaaacctatgagtgttggtcttgggttgaggccaaggtactgcctttgagttggagacttgtcggccagtgctgaggctattctcctggcagttggagtctgagcatggctaggagcccccactggtccaaaccttctaagcccataggtgtaaggcagcactgatgtgaggaggtgcacaggtttgttttcattctgtattaacttcctgaggcagctctgccatggcctgtgtcagaagcttgggtctagaggtggcgcagccattatctgtgtcataggtggcagcatatggacacatgtatgtacacctgtgtgcatatgcatggatgtgagtgcaaggacacacggtgccaattcagaacaatgacatgaaggtcagaaggggccatgtctatattcagagagaacccagaggaggaagagcctacattaggcccaggagagtagagggtacttctgggagaaggaagacctcagccacaaggacagagggacagatggacagacatcctaaaaagagaagctttgtgtggaggtccttgtcacagtgagtcaagccactgtcttaaaaaaactacatcttctcagagccttgctgggtctcacccagcaggcaggagggaagccctaaagtaacccacttcctggcccagcaaactgcagacacaagcgtgccacgctgaagaggaaggccaagaagggaaaaagcctgggctctactctctcaagccttcctcgtcctccaacgcaaaaacccatccatgaggcctggtgacaggtatgctggagcccagagtcatactgatggctgcctcccttgttcccttccaggttgtcttgacaccctacaaaccggaacctgggtacgagtgccagatctcacaggaatactatgacaggaaggctcagatgtgctgtgctaagtgtcctcctggtgagaggcagctgctggggctttggaaggtggtgccatggagggagtgcttgtctgggaatgagggccttcagctctcactggctgctttatacatgctagggttcatgattcatcttgccctgggctcttgcatgtgctgtgccctccactgagcacacttctcagtgtcttctcctggttactgcctacctacattttgaccctatcctcttgtccaggaagcctcctcaatactgcaatgatgtcctagtacttttcatagccccactatgtgctatgtctacccctattgagtagtgagtgtagcttggtccctgtggagttccaagcacacggctggcctatattgatgtcctgtacttaattgtcaagtaaatgaatggatagccatatcatagatggcggatctgagccctggcctcattggcgaggactgagtagctggcccccagtgctgagtagacaatcaagtgtatgcattcaattaagtcgtatttataatgcatctactctgtgctcaatctgctgagaggaaagccacacaaacacgggatacagcaggctgggaagtaagtgcaaagccctaaagcaggggcctgttttaatgggtccaaagaagcttgaggctggtgtttgttgcccagagtgaaagaagagtgtgatggaagatgggtatgaaggggtgagggttggtgagatggctctgtatgtaaaggcacttgctgtgcaagcctgagaacctgaaccaatggtggaaggagaaaacaggttacacacacacaccaccaccaccaccaccaccaccaccatcgtaataatatacatttgattaagcgagatgagtggtgtcaccatgaagaattcagatttcatttactggaggctttgagtcctgtgcttgtgacccagtgggcaggaacacagggcaatgtcatcctccacagtcacagccaggggacagtggcttttctagtgacgagcagagtgtctttacgaagttacaagcttagagtagcaggaacagaggagacgagctggttccagaagagaaaaccttaaagatttgtcctgttactcttctatcctccaggctcttaggagccctatgcccttggcactgacaggctaccagacatgacgcccttatagccacttatatttagtacatcaggatagagaattttaaccaactatcaagaagacaggagctagcaaacccattctcccttaagtattcttgactgttaataggtttttcgagtggtggtgtttcaactacctggagagagcagagggaagatatgttcagaggtagagagatagctagggccaccagacatgcttcatcccaggggcttcctggcaagggtcttctgctgagacctctggtccttgcttcctcaggccaatatgtgaaacatttctgcaacaagacctcggacaccgtgtgtgcggactgtgaggcaagcatgtatacccaggtctggaaccagtttcgtacatgtttgagctgcagttcttcctgtaccactggtgagtggcatgagcactgtgatcccaacatcttccccagtcactcgccgtccagcaagtaaggtggatggggttaccctgggccagccgttttcgtcttccaggacttgagttgcgggagactgctttttttaaaatatttttttattacatattttcctcaattacatttccaatgctatcccaaaagtcccccacaccctcccccccactcccctacccacccattcccattttttggccctggtgttcccctgtactggggcatataaagtttgcctgtccaatgggcctctctttccagtgatggccaactaggccatcctttgatacatatgcagctagagttaagagctccggggtactggttagttcataatgttgcacctacagggttgcagatctctttagctccttggatactttctctagctcctcccttgggggccctgtgatctatccaatagttgactgtgagcatccacttctgtgtttgctaggccccagcctagtctcacaagagatggctatatcacggtccttgcaccaaacgcttgctagtgtatgcaatggtgtcatcgtttggaggctaattatgggatggatccctggatatggcagtctctagatggtccatccttttggggagactgctttttttcaacttgtatgtagttatgtgattggaacctgggacttcatgcaggtgatgcaaacacttttttttttttttttggttttttgagacagggtttctctgtgtagccctggctgtcctggaactcactttgtagaccaggctggcctcgaactcagaaatctgcctgcctctgcctcccaagtgctgggattaaaggcgtgcgccaccacgcctggctgatgcaaacactttttaacagaactacatcaatccccagatattttttttattaaaggtgtattaattaattaattaattaattaattaattaacttacttattttggtttttcaagacagcatttctctgtgtatcctcggctgtcctggaagtcactctgtagaccaggctggcctcgaactcagagatctgcctgactctgtatcccaagtgctaggactaaaggcgtgcgccgccccaacccaataagatttatttatttttattgtatgtatatgggtatttttactggcatgtagtcaggatctattttgccttgagtcaggatctctctaggtagctcagaatggctttgaagttatgaactgcctaactcagcttcctgagtagctgagaatacagacctgaactcccagaaaatgttttcagttcagatttttttgtttgtttggtttttgttgttattgtatttgtttatttggttttggtttttataagatagggatgtgtgtgtgtgtgtgtgtgtgtgtgtgtgtgtgtgtgtatatagtcttggctgttttgaaactgaactaactctgtagaccaggctggccttgaactcatagagctccaactgcctctgcctcctgagtgctgggattagagatgtatgccacccctgttttttgttttttgggttttgttttttttttttttttgagatggtttttttgctaagttgcccaggttggcctagaactttctataaggcccaggctaactttaaatttacattcatccttctgcctcggtttccccagtgttgagattacaaatgtgtgacacctgcctggacagttccagatgacattttccttctagatcctaccaaatcttcattggtagtggggaggtgaggtcagagttgagaatgtagagcctagagaaacagatgtgtatattcactctgtggtggagttcagagtacagacaacaacagcccaagaggcaaggtgttcaagggtcctttgggcctgtgctgagggccctaccagctctggcaggaagagcagaatgggtgagtggaagtagagatgaccctggctgtctttctcacctctagaccaggtggagatccgcgcctgcactaaacagcagaaccgagtgtgtgcttgcgaagctggcaggtactgcgccttgaaaacccattctggcagctgtcgacagtgcatgaggctgagcaagtgcggccctggcttcggagtggccagttcaagtaaggatccctcttcctctccctgggaaaggatgtgaacatccctgagatgtcacaggcacttacctctctaagccttacctctaagcctccagtagctgccacatgcattacatgtctcctggcacccctggttacaccaagcccttagctagtaggaaatcaggtaggacaggaaggtaaccctggacagcaagtccatgtacatgtatggtcatgtgtgtccatgcatgcatgcatgcgcgcgcgcgcgcgcgcgcgtgtgtgtgtgtgtgtgtgtgtgtgtgtgtgtgtgtgtgtgtgtgtgtgttttaagggagaggattacaaagtggcctcccttgtggccccactgttaagagactccccacctggctacatgaagtgttcatattgtcgacaagctctggattttctcttcaaggagccccaaatggaaatgtgctatgcaaggcctgtgccccagggacgttctctgacaccacatcatccactgatgtgtgcaggccccaccgcatgtgagtgttgacttcctggcttctgaaggagcagggagggtgaccgcctaggggaactgggtcccaggatataggacagcttgtcactctttgtctcttgacttgggttctgggacagacaatggatgacttgagcaggaacctgacatagaggcaagattggatagagtgacactgggtggaagttgaggagtatatgagggggtagtgctaagaagcccatactcattgcttggctgttaggatccttgtcctcaggcctggctccctgaaattctgtggtcttctatcttctgtggtctcctgattacaatcttcctcccccagctgtagcatcctggctattcccggaaatgcaagcacagatgcagtctgtgcgcccgagtccccaactctaagtgccatcccaaggacactctacgtatctcagccagagcccacaagatcccaacccctggatcaagagccagggcccagccaaactccaagcatccttacatcgttgggttcaacccccattattgaacaaagtaccaagggtggcatctctcttccaattggtaagtcctcagtctcaagagtgacccaggcaggcttggaagtgtgcagtctgagctactggggaagctgagacaagagaattgcaagttcaaggccaacctgggctatagagtaagtttgaggtcaatctgggcaacttagtcagaccctgtctcaaaatagtacttttaatgggagctgaggctgtagcccattggtagaatgtctgactagtttggggttaaatctgtaacaaaagtaaattgaaacataaaagggaggtgatcccccacccccaccccctgtctctcttgcctccctttgggcagaactggggcctggtctctgtcttttagaacagatgcaagtgtagaagagttgagtctccaaagatgtgatattgccatagggaatccctgggtggcatgaatgtgaacataggttctggttgctagttatgatgaacccgtttgtctcacagactatggactgctggtgtctctggcttccctctggggttaggatggtaccaagcccaaggccctacactgtagccttctgactgcatgtggtttgcagatgtgatctttggtttgaccctgaatttgagggcctaaggctggacttgatctcagcatcagcaccagccaccctggaacctttgtttctgagtaccctgccgttttcctaggtctgattgttggagtgacatcactgggtctgctgatgttaggactggtgaactgcatcatcctggtgcagaggaaaagtaaggttctgctctcgtcctgtttcccgccccacgtccctaccctaacactttctcggagccttgggtggcaggcctcgttcagagctctgcactatcatagactcgggtggatctggagactgtagcctcttgctctccaggaacttagagcctggtgtagaaggtacatactctaacctggctaccagaaggtagtgtcaaggctattccaggggattgaagttcaggatttttatacaggaagcctggagtctctcggattctgtgagctggcctgggtctcagtgggtggagtgtgttgaggcagggctacaacacaggctgtactggaggatggctggggcaaaggggtagtggctgaaagtagcatgggctcatccgtgaacatgacaggcagctactccctgggctgggtccactctcctggctctaccctagccatgctgtgcccattaagacagctgttctgaagaagtcctgcctctgacttgttcccctctcttcattgtagagaagccctcctgcctacaaagagatgccaaggtggtgagtatccctctgcggtcctcctcccccttctctcctccagctctccctcttcctcctcctctttctcctcctcttccagttcctttactagggcatcataagcaacatcatataagcaggatctaatgtatatggtggtgcatacctgccatcccaatagttaggggcaggtagaggctggagggtcagagtgtaaatactccctcagagccagctgatgtttagttccattacagttgggaagaaaccggcaaactctcccctagctgggcatagccaggctctttccctaggctatgtccaactcctcactggtcctatgcataaggcaccttggctcctcattatatagatgaggaaatgtaggcttaacagatacagtcacccttgaaaggttgtgttgtgtcctggtggtcaaaccctctgcgcatgtgcatccggcagctacacccaaagctgtctcaggctggcctctcctagcagggactgctcgccaagactggtcaccaggatttggagaacctagatgcccccctttgtccagccctgtgccctgtcagctacctgccccagggccctactctggagcccagtggacggtgtcctcatgtgctagagtgaggaggctgtcaggcaggagcagcagtgactcagcttctactctgaggactggggaagatgaggttatctggaaaaacagcacgtgaattcatctacacctcccccagtcatgcgcatggttcatgtttagtcgccggcagttactggtggtggtggaggaaggacgtgccagcactgtctgagggcttattcttccagcttgactgtgacacaggctatgacacaggctgtggcacaggctgtgacagaggttattgcccccaacgttagacagagtctgggattatatggctcagacactcttaagtaattgtcctgtgtcctagctgtgtcctagacacagctaatgggtatggcctggaacacaaacttagcatacaattactacccagcatacaattactgtgccactcttaggcatgcccacatgagcctgcacatataaatacccttagctcagaggccgacagaagccagccatgcttctgccagtcccagttccatataacaggaccagacccagaaccataggaggtatcaggcaagctaagattttttggtgttcattcagtggggtcctagccagagtcacatgactctgatagtgtctgtacttgaacactgtagcttgtggctttgaagaagctagctgtgacctttggggaggaggggaagatcgggttctgtctggctctagccacaagcagaaagggggaggcccagacagaaaagctccttctctggggctggtgtggtgtgacatttatgagtgcctctgtagagttacagggtaaggccagggccaaggtcagaccgtgagttcaggatgtttttcctctcttccattttggggtacctagctgggaggaccccaggggagtcaggaggatgcagtgggcatgctcccacatcctagactgggtttgcttactgtggccatcagccagctctgtaactctgagctctggattcatcttctgtgggcttttgtggcctcatgaagacagcttgtataagatccttccagtccagagtcagaagctgtggactgtgcaggaaacaaggcctcaaggccatgtatcatgacatacctgggcatctaagaagacatagcaacagtgggcaggacctggagatggaagttttagtgactctctagagagcaccagccacaggaaggatagcccaactattgtttcagcttagactacacctggcattgtgcctccctggaaaagtgtggccacttttccagctgctgtcaacagacaatggccttggaatagatgtccttagcataagttgccatgaacagggaatttgtcttaagcctcaagagctgaaccccagacacccagaagaggcatggtgagtttttagctcgactgcactgtatccaaaccatggcctcaggcagaaagttccgtttccatatttacagagctaggatggcactaggctatattgagtgtctagaagagctgagaccaatgtgactcaggcacaggatttggcactaggtgctcatgtcacatacagagtaagaagccacagggaagccacacgacatcatctgggtgaactgtgggaacgggcagctgagaagaccagtgaggaaccctgtgagtggccctgtgagtggccctgaggaaaggaccccatgggccagggtgattcattgagcagaaggaatgaagagtaaaggtgttaagcttcaagcaccaaggctggcctctgggacagctactctgatctgccacccaccatcaggaagtctgtgctttgcaaaacattgatgacagctcaggtgcatcaaacttgtttatttacgaacactaaaacttgacctttagatttgaggcattttgtattttagacacggacttatgtagcctgtattgaccctgaacactaactgaggatggctttgaatttatgatcctcctgcctcaacctccccagtgctgggattactacatacaccaccacaccctgcttgtgtgatgctggggactgaacccctgagctctaggcagagtctttagtcccttctgttcttgcagaaaacatgatttcagttctcagcaccaagagaggttaggtaactttttcaaggtcatctagccagtgagtggtagagctatgaactttagactcaggtgtctggttcagaattcatctcttagctgccaggctggtgacacatctccctatgctccaaaaagtcactttttccatttccttgtgaggactgagattgaaaacctttggtgccctgtgtggaaacgtgtggtgtgggcagaaatgtgtaagctgtggagtgtgggtgacaggggagactaggagagcaaaggcacttgcagatggattaatattctctcttttcctcccagcctcatgtgcctgatgagaaatcccaggatgcagtaggccttgagcagcagcacctgttgaccacagcacccagttccagcagcagctccctagagagctcagccagcgctggggaccgaagggcgccccctgggggccatccccaagcaagagtcatggcggaggcccaagggtttcaggaggcccgtgccagctccaggatttcaggtgagaggctgattccctcctgctctggacagatagctggccctccacctactggttgaaaataacccaagaggaaaatgcctttaacacttggtggctatgacaacggacagaatggctctgatctgctgcccagtgtcttgcgagaggatcctattgcaattcaatagttccgaaaaaggtccaggctcacagtgctaaacacagctcccatggaatgcgtgtatcatgttcccaccaacgtcaagttgcaaaacctcgagtcagacttctgtaggtaaagtcaggttcatgtgtatcccttgcgtaatctctgctggtgtcctggagctgccctgtgaagccacccttagctgagcctggctgacttcctagttctggctcatgtgcagtccagccacggtaggttcagcgccacctgtgttggttatctcactagctcattcgtcttcagacacccctgctttgtctttcaaggcttccatatcaggtggggagtaatcctgaacccctccacgttgtcatctctggccagcttggcctttgttcagggatccccaaggtcatgccgcctttccacaggattatctgtcttctgcctttcgatggcctgtgtgatttccccaaagccacgttctgcttatatccctaggcccagcactggtctggctagattgtttgtttgtttgtgagacaaggtttctctgtgtagcctaggctgtcctggaacttgctttgtagaccaggctggcctggaactcagagctccctctgcctttgcctcctcagtactgggattaaaggcatgtgccaccatccctcattggcctgtccagttttataagctaatacttcctagggcattgtaacacaccagtctttgtcctgggtgctttacatgaaccaaacctgcctatcaatactaagagatagttactattactaccccattttccagatgaggaaattgaggtccaggacaccttgttaagaggacatagctagtgcacccaagctccaggagtcatcagctctgcagtatgagcttcagagccctggaaatgggagatgaatgaaatagttccttcagggttctttaaaaatgttttgtgtatgggtattttacctgcatgcatttccatgtactgtaggtgtgcatggtgtctatagaggccagaagagggtgtcagatctcctagaaatggagttacagatggttgtgaagtgccatgtgggtgttgtgaatctaacctaactcctctgaaggagcaacaagtgctcttagctactgagccacctctccagacccattcttctgggggttctgctcactgtagctcactgatgatgatcactttgagtcaaaggcatgatgtgtgaccctgttgcctttacttggtctgcatcttaccctacatatatataatctataatagagacactattggtatctcttgtgcctacaatggagtcagtcccttgtaggtttcccaagaacccagagattccctttggtttggtttgtagaagaaagggcaagactacaggcctttgtccctctctcccggcagcacaggcgagtggggcaataggaagtataaacatgaacgtgaacttggtcattcacccagagcagcccaacagccctggggccatgagaatccaagcaggctcctacatcccatttcctcatctggtgatgagacatgctcttccttagcacgtcaatgagagactgtggctttgtgcccacattggctcctgacaggggattgacagccaagaccacactgcctcccacaccagcctcctctaacacccatgttctgttgctgccttgacttccgtgccctgctcttactcctgcctattcaagcttttctgcctgcagcactcctgctgtctccctgcccgcaggagtcccggtgtctgctttgtgtttttcccgtcggaaccccagcctcactagcacgtggtaacttgtcagggcccctggctctgacctgaggattccctgagcctggcttggaacagaacaggtgtctcttaacattggttgagtgaatacatgtgcttgaatagaagcatgaattcatctttcatggcttccctcctcccatggtgttccactgtggctccttctttggtccctgaggacctaagttctttctcctctgacctctgccccctcctctttcttctcccaggtgtactgtacctctcctcctctcccattgacacctccctctacccgtggggcctgtaaaccccagaattgccccactcacccccacatgttcatgacatgcaaaggtcatggtgacttcaaatgacgttcgggtgctgttgaggcccagggtagaggtttctttgtggtcccttgattccagttctccctctgcttgatatatttgaggctgctctgaatagactggttggctctgtcctaacccaagctcccttgagtcccaatttccgggaggcagaagccaggataaatagacagctgccactactatgggccccggggggttctgcagatctagctgcagtcgcaagagcaattgccatgcagttgacatttgggagtaacatatgtctaccctctgctagtctggcattcactcctcgccaacttagagaacttagaagcccacagaggtcaggcaggatgatagatggactgtccctgatattcgttctgtctgtgatttctgcttctctatatcccagtggtagggatcaaaatccacgtgtctggtaggtgagctttaaactgccaacccctaaattttaagtgttgtcagtcaattcacttaaaatgctatcatcaccaaaaccaaagtgtgcctaggctggttttgatccatttggtacttgccctttcagtggtcatggggaatattctttgtagatttggccataggcagtcttctgtaactgcttcctgccacatcctagcttctctgttccagcaaactgctctctctctctctctctctctctctctctctctctctctctctctctcacacacacacacacacacacacacacacacacaggtgtgctaatgagtccacgtgtctatgtggaagctagaggacaacctcaggtggcatccttaggaaccccatctgcctcctttaagacagtttccccttggcttggtgtccaccagttagacttagttggttggcctgaaaagacccagaaatctccctttctctgcctcccaagtactgagattacaagtgtgtgccgccatgcccagcctccttacatggggtctcaggggttgaatttaggtccttaagcttgcaagacaaagtccttactaactgagccatatcctcagcccaatgttttgttcttcttggagtacttttgtctgctttagaaaattgtctccggtcaacagcagggagcgttgggctgggcagctgggaagtgagcacacaggcatgtaagggtgatgcatctgccatcgtagtagaggtgagctagggtctttagcctcttggcccttggcctattgctctaacctgcccctgggacaagaggcaaactgcaaagacaccctgtctccaagatccccagactcaccctcccatcctgtgcttcacagattcttcccacggaagccacgggacccacgtcaacgtcacctgcatcgtgaacgtctgtagcagctctgaccacagttctcagtgctcttcccaagccagcgccacagtgggagacccagatgccaagccctcagcgtccccaaaggatgagcaggtccccttctctcaggaggagtgtccgtctcagtccccgtgtgagactacagagacactgcagagccatgagaagcccttgccccttggtgtgccggatatgggcatgaagcccagccaagctggctggtttgatcagattgcagtcaaagtggcctgacccctgacaggggtaacaccctgcaaagggacccccgagaccctgaacccatggaacttcatgacttttgctggatccatttcccttagtggcttccagagccccagttgcaggtcaagtgagggctgagacagctagagtggtcaaaaactgccatggtgttttatgggggcagtcccaggaagttgttgctcttccatgacccctctggatctcctgggctcttgcctgattcttgcttctgagaggccccagtattttttccttctaaggagctaacatcctcttccatgaatagcacagctcttcagcctgaatgctgacactgcagggcggttccagcaagtaggagcaagtggtggcctggtagggcacagaggcccttcaggttagtgctaaactcttaggaagtaccctctccaagcccaccgaaattcttttgatgcaagaatcagaggccccatcaggcagagttgctctgttataggatggtagggctgtaactcagtggtccagtgtgcttttagcatgccctgggtttgatcctcagcaacacatgcaaaacgtaagtagacagcagacagcagacagcacagccagccccctgtgtggtttgcagcctctgcctttgacttttactctggtgggcacacagagggctggagctcctcctcctgaccttctaatgagcccttccaaggccacgccttccttcagggaatctcagggactgtagagttcccaggcccctgcagccacctgtctcttcctacctcagcctggagcactccctctaactccccaacggcttggtactgtacttgctgtgaccccaagtgcatgtccgggttaggcactgtgagttggaacagctgatgacatcggttgaaaggcccacccggaaacagctgaagccagctcttttgccaaaggattcatgccggttttctaatcaacctgctcccctagcatgcctggaaggaaagggttcaggagactcctcaagaagcaagttcagtctcaggtgcttggatgccatgctcaccgattccactggatatgaacttggcagaggagcctagttgttgccatggagacttaaagagctcagcactctggaatcaagatactggacacttggggccgacttgttaaggctctgcagcatcagactgtagaggggaaggaacacgtctgccccctggtggcccgtcctgggatgacctcgggcctcctaggcaacaaaagaatgaattggaaaggactgttcctgggtgtggcctcagctcctgtgcttgtgtggatccctaaagggtgtgctaaggagcaattgcactgtgtgctggacagaattcctgcttataaatgctttttgttgttgttttgtacactgagccctggctgagccaccccaccccacctcccatcccacctttacagccactcttgcagagaacctggctgtctcccacttgtagcctgtggatgctgaggaaacacccagccaagtagactccaggcttgcccctatctcctgctctgagtctggcctcctcattgtgttgtgggaaggagacgggttctgtcatctcggaagcccacaccgtggatgtgaacaatggctgtactagcttagaccagcttagggctctgcaatcagaggagggggagcagggaacaatttgagtgctgacctataacacattcctaaaggatgggcagtccagaatctccctccttcagtgtgtgtgtgtgtgtgtgtgtgtgtgtgtgtgtgtgtgtgtccatgtttgcatgtatgtgtgtgccagtgtgtggaggccagaggttggctttgggtgtgtttgatcactctcagttactgaggcagggctctcatctgtacccagagcttgcacattttctagtctaacttgcttcagggatctctgtctgcctatggagtgctcaggttacaggcaggctgccatacctgcccgacatttacatgaatactagagatctgaattctggtcctcacacttgtatacctgcattttatccactaagacatctctccaagggctcccccttcctatttaataagttagttttgaactggcaagatggctcagtgggtaaggcagtttgcggacaaacctgatgacctgagttggatccctgaccataaggtagaagagacctgattcctgcaagttgtcctctgaccaccaccccatacatgcttctgcatatgtgcacacatcacattcttgcacacacactcacataccataaatgtaataaatttttttaaataaattgattttatcttttaatcattatttttgcttatctgtttgttcatacatggagttttgctgtatacccagtctggctgcatcctccaggcaccttgaacttggatattctcctgcctcagtttcgagagtgctgagttataggcatgtgcaaccgtgtcaggacccttggcgttacattatgttttcgaatcttatttttccatctaagactgacaaccaccttgccaaaggatgaccttgacttttgtatcctcttgcctctacttcccaagtattgggatgacaagtctgtccatcctatgatttgtgtggtgctggggcttgaacccaggggcctcgtgaatgctaggcaaacgcaatcagctgcccaaccccgaacttcacttttcacctgtgatttcttaacatggttcctgagcagacagcatgatcctgttgccttgaggagctctgctcgttgctttgacaatgctctatttactaaagaatacttatagagttcaagactccaaagcagcagttcccaacctgtgggtatgacctcttgggtatcccatatcagatatttacattaaacttataacagaagcaaaattacagttatggggtagcaacaaaataatttttttttgaggcagggtttatctgtgtagctcactttgtacagactaggctggccttgaacttaaagatctgcctgcctctgccttctgaatgctgggattaaatgtgtgtgccaacatgcccagtgcagtgaaataattttattgttgggtcaccaaaacatgagaaagagtattaaaaggtcatagcgttaggaaggttgagaaccactgccccaaaagatagtagaaataggtaatagcattttaaaaaaagattaatttctttttccgtgtgtgtgtgtgtgtgtgtgtgtgtgtgtgtgtgtgtgtgtgtgtgtgtgtgtgaagggtgctgaattccctaaatctgggattacagacaattgtgccaaatgggtattgggaaccaaagttgggttttctgaaagagcagcaagtgcccttaactgctgagccctctctctagctataataaacttttttttaaaaaaattaaaaaaatttagcactc

SEQ ID NO: 16 - DNA, 4913 bp, Mus musculus
  source 1..4913: mol_type = genomic DNA
agtcaccagctagagcgcagctgaggcactagagctccaggcacaagggcgggagccaccgctgcccctatggcgcccgccgccctctgggtcgcgctggtcttcgaactgcagctgtgggccaccgggcacacagtgcccgcccaggttgtcttgacaccctacaaaccggaacctgggtacgagtgccagatctcacaggaatactatgacaggaaggctcagatgtgctgtgctaagtgtcctcctggccaatatgtgaaacatttctgcaacaagacctcggacaccgtgtgtgcggactgtgaggcaagcatgtatacccaggtctggaaccagtttcgtacatgtttgagctgcagttcttcctgtaccactgaccaggtggagatccgcgcctgcactaaacagcagaaccgagtgtgtgcttgcgaagctggcaggtactgcgccttgaaaacccattctggcagctgtcgacagtgcatgaggctgagcaagtgcggccctggcttcggagtggccagttcaagagccccaaatggaaatgtgctatgcaaggcctgtgccccagggacgttctctgacaccacatcatccactgatgtgtgcaggccccaccgcatctgtagcatcctggctattcccggaaatgcaagcacagatgcagtctgtgcgcccgagtccccaactctaagtgccatcccaaggacactctacgtatctcagccagagcccacaagatcccaacccctggatcaagagccagggcccagccaaactccaagcatccttacatcgttgggttcaacccccattattgaacaaagtaccaagggtggcatctctcttccaattggtctgattgttggagtgacatcactgggtctgctgatgttaggactggtgaactgcatcatcctggtgcagaggaaaaagaagccctcctgcctacaaagagatgccaaggtgcctcatgtgcctgatgagaaatcccaggatgcagtaggccttgagcagcagcacctgttgaccacagcacccagttccagcagcagctccctagagagctcagccagcgctggggaccgaagggcgccccctgggggccatccccaagcaagagtcatggcggaggcccaagggtttcaggaggcccgtgccagctccaggatttcagattcttcccacggaagccacgggacccacgtcaacgtcacctgcatcgtgaacgtctgtagcagctctgaccacagttctcagtgctcttcccaagccagcgccacagtgggagacccagatgccaagccctcagcgtccccaaaggatgagcaggtccccttctctcaggaggagtgtccgtctcagtccccgtgtgagactacagagacactgcagagccatgagaagcccttgccccttggtgtgccggatatgggcatgaagcccagccaagctggctggtttgatcagattgcagtcaaagtggcctgacccctgacaggggtaacaccctgcaaagggacccccgagaccctgaacccatggaacttcatgacttttgctggatccatttcccttagtggcttccagagccccagttgcaggtcaagtgagggctgagacagctagagtggtcaaaaactgccatggtgttttatgggggcagtcccaggaagttgttgctcttccatgacccctctggatctcctgggctcttgcctgattcttgcttctgagaggccccagtattttttccttctaaggagctaacatcctcttccatgaatagcacagctcttcagcctgaatgctgacactgcagggcggttccagcaagtaggagcaagtggtggcctggtagggcacagaggcccttcaggttagtgctaaactcttaggaagtaccctctccaagcccaccgaaattcttttgatgcaagaatcagaggccccatcaggcagagttgctctgttataggatggtagggctgtaactcagtggtccagtgtgcttttagcatgccctgggtttgatcctcagcaacacatgcaaaacgtaagtagacagcagacagcagacagcacagccagccccctgtgtggtttgcagcctctgcctttgacttttactctggtgggcacacagagggctggagctcctcctcctgaccttctaatgagcccttccaaggccacgccttccttcagggaatctcagggactgtagagttcccaggcccctgcagccacctgtctcttcctacctcagcctggagcactccctctaactccccaacggcttggtactgtacttgctgtgaccccaagtgcatgtccgggttaggcactgtgagttggaacagctgatgacatcggttgaaaggcccacccggaaacagctgaagccagctcttttgccaaaggattcatgccggttttctaatcaacctgctcccctagcatgcctggaaggaaagggttcaggagactcctcaagaagcaagttcagtctcaggtgcttggatgccatgctcaccgattccactggatatgaacttggcagaggagcctagttgttgccatggagacttaaagagctcagcactctggaatcaagatactggacacttggggccgacttgttaaggctctgcagcatcagactgtagaggggaaggaacacgtctgccccctggtggcccgtcctgggatgacctcgggcctcctaggcaacaaaagaatgaattggaaaggactgttcctgggtgtggcctcagctcctgtgcttgtgtggatccctaaagggtgtgctaaggagcaattgcactgtgtgctggacagaattcctgcttataaatgctttttgttgttgttttgtacactgagccctggctgagccaccccaccccacctcccatcccacctttacagccactcttgcagagaacctggctgtctcccacttgtagcctgtggatgctgaggaaacacccagccaagtagactccaggcttgcccctatctcctgctctgagtctggcctcctcattgtgttgtgggaaggagacgggttctgtcatctcggaagcccacaccgtggatgtgaacaatggctgtactagcttagaccagcttagggctctgcaatcagaggagggggagcagggaacaatttgagtgctgacctataacacattcctaaaggatgggcagtccagaatctccctccttcagtgtgtgtgtgtgtgtgtgtgtgtgtgtgtgtgtgtgtgtgtccatgtttgcatgtatgtgtgtgccagtgtgtggaggccagaggttggctttgggtgtgtttgatcactctcagttactgaggcagggctctcatctgtacccagagcttgcacattttctagtctaacttgcttcagggatctctgtctgcctatggagtgctcaggttacaggcaggctgccatacctgcccgacatttacatgaatactagagatctgaattctggtcctcacacttgtatacctgcattttatccactaagacatctctccaagggctcccccttcctatttaataagttagttttgaactggcaagatggctcagtgggtaaggcagtttgcggacaaacctgatgacctgagttggatccctgaccataaggtagaagagacctgattcctgcaagttgtcctctgaccaccaccccatacatgcttctgcatatgtgcacacatcacattcttgcacacacactcacataccataaatgtaataaatttttttaaataaattgattttatcttttaatcattatttttgcttatctgtttgttcatacatggagttttgctgtatacccagtctggctgcatcctccaggcaccttgaacttggatattctcctgcctcagtttcgagagtgctgagttataggcatgtgcaaccgtgtcaggacccttggcgttacattatgttttcgaatcttatttttccatctaagactgacaaccaccttgccaaaggatgaccttgacttttgtatcctcttgcctctacttcccaagtattgggatgacaagtctgtccatcctatgatttgtgtggtgctggggcttgaacccaggggcctcgtgaatgctaggcaaacgcaatcagctgcccaaccccgaacttcacttttcacctgtgatttcttaacatggttcctgagcagacagcatgatcctgttgccttgaggagctctgctcgttgctttgacaatgctctatttactaaagaatacttatagagttcaagactccaaagcagcagttcccaacctgtgggtatgacctcttgggtatcccatatcagatatttacattaaacttataacagaagcaaaattacagttatggggtagcaacaaaataatttttttttgaggcagggtttatctgtgtagctcactttgtacagactaggctggccttgaacttaaagatctgcctgcctctgccttctgaatgctgggattaaatgtgtgtgccaacatgcccagtgcagtgaaataattttattgttgggtcaccaaaacatgagaaagagtattaaaaggtcatagcgttaggaaggttgagaaccactgccccaaaagatagtagaaataggtaatagcattttaaaaaaagattaatttctttttccgtgtgtgtgtgtgtgtgtgtgtgtgtgtgtgtgtgtgtgtgtgtgtgtgtgtgtgaagggtgctgaattccctaaatctgggattacagacaattgtgccaaatgggtattgggaaccaaagttgggttttctgaaagagcagcaagtgcccttaactgctgagccctctctctagctataataaacttttttttaaaaaaattaaaaaaatttagcactc

SEQ ID NO: 17 - protein, 474 aa, Mus musculus
MAPAALWVALVFELQLWATGHTVPAQVVLTPYKPEPGYECQISQEYYDRKAQMCCAKCPPGQYVKHFCNKTSDTVCADCEASMYTQVWNQFRTCLSCSSSCTTDQVEIRACTKQQNRVCACEAGRYCALKTHSGSCRQCMRLSKCGPGFGVASSRAPNGNVLCKACAPGTFSDTTSSTDVCRPHRICSILAIPGNASTDAVCAPESPTLSAIPRTLYVSQPEPTRSQPLDQEPGPSQTPSILTSLGSTPIIEQSTKGGISLPIGLIVGVTSLGLLMLGLVNCIILVQRKKKPSCLQRDAKVPHVPDEKSQDAVGLEQQHLLTTAPSSSSSSLESSASAGDRRAPPGGHPQARVMAEAQGFQEARASSRISDSSHGSHGTHVNVTCIVNVCSSSDHSSQCSSQASATVGDPDAKPSASPKDEQVPFSQEECPSQSPCETTETLQSHEKPLPLGVPDMGMKPSQAGWFDQIAVKVA

SEQ ID NO: 18 - DNA, 20 bp, synthetic construct
  misc_feature 1..20: note = gRNA sequence
  source 1..20: mol_type = other DNA
cggacagtcactcaccaagt

SEQ ID NO: 19 - DNA, 22 bp, synthetic construct
  misc_feature 1..22: note = Single strand DNA oligonucleotide
  source 1..22: mol_type = other DNA
gaacaattccatctgctgcacc

SEQ ID NO: 20 - DNA, 21 bp, synthetic construct
  misc_feature 1..21: note = Single strand DNA oligonucleotide
  source 1..21: mol_type = other DNA
ttcgaaatcctgacctcctgg

SEQ ID NO: 21 - DNA, 20 bp, synthetic construct
  misc_feature 1..20: note = gRNA sequence
  source 1..20: mol_type = other DNA
gacactgcctgaggtaattc

SEQ ID NO: 22 - DNA, 22 bp, synthetic construct
  misc_feature 1..22: note = Single strand DNA oligonucleotide
  source 1..22: mol_type = other DNA
tgagacagggtttctctatacc

SEQ ID NO: 23 - DNA, 18 bp, synthetic construct
  misc_feature 1..18: note = Single strand DNA oligonucleotide
  source 1..18: mol_type = other DNA
catggcattcgtctttgt

SEQ ID NO: 24 - DNA, 20 bp, synthetic construct
  misc_feature 1..20: note = gRNA sequence
  source 1..20: mol_type = other DNA
cggcttcccagaattacctc

SEQ ID NO: 25 - DNA, 20 bp, synthetic construct
  misc_feature 1..20: note = Single strand DNA oligonucleotide
  source 1..20: mol_type = other DNA
agtgagagcagagaattgtc

SEQ ID NO: 26 - DNA, 20 bp, synthetic construct
  misc_feature 1..20: note = Single strand DNA oligonucleotide
  source 1..20: mol_type = other DNA
gagcttgcatgtgcacgcat

SEQ ID NO: 27 - DNA, 20 bp, synthetic construct
  misc_feature 1..20: note = gRNA sequence
  source 1..20: mol_type = other DNA
atatacccctcaggggttat

SEQ ID NO: 28 - DNA, 22 bp, synthetic construct
  misc_feature 1..22: note = Single strand DNA oligonucleotide
  source 1..22: mol_type = other DNA
tctcacactccctgcagtccgt

SEQ ID NO: 29 - DNA, 22 bp, synthetic construct
  misc_feature 1..22: note = Single strand DNA oligonucleotide
  source 1..22: mol_type = other DNA
cagattgtatggccccaactgt

SEQ ID NO: 30 - DNA, 20 bp, synthetic construct
  misc_feature 1..20: note = gRNA sequence
  source 1..20: mol_type = other DNA
attggactggtccctcacct

SEQ ID NO: 31 - DNA, 21 bp, synthetic construct
  misc_feature 1..21: note = Single strand DNA oligonucleotide
  source 1..21: mol_type = other DNA
ttctgaagcggtgaaggagcc

SEQ ID NO: 32 - DNA, 22 bp, synthetic construct
  misc_feature 1..22: note = Single strand DNA oligonucleotide
  source 1..22: mol_type = other DNA
cagattgtatggccccaactgt

SEQ ID NO: 33 - DNA, 20 bp, synthetic construct
  misc_feature 1..20: note = gRNA sequence
  source 1..20: mol_type = other DNA
tacttgtacaatgactgtcc

SEQ ID NO: 34 - DNA, 21 bp, synthetic construct
  misc_feature 1..21: note = Single strand DNA oligonucleotide
  source 1..21: mol_type = other DNA
tgccggtactggttcttcctg

SEQ ID NO: 35 - DNA, 22 bp, synthetic construct
  misc_feature 1..22: note = Single strand DNA oligonucleotide
  source 1..22: mol_type = other DNA
gggtgctgcttctttctctgct

SEQ ID NO: 36 - DNA, 20 bp, synthetic construct
  misc_feature 1..20: note = gRNA sequence
  source 1..20: mol_type = other DNA
taatgtatcgctaccaacgg

SEQ ID NO: 37 - DNA, 17 bp, synthetic construct
  misc_feature 1..17: note = Single strand DNA oligonucleotide
  source 1..17: mol_type = other DNA
accacagtgctgttgcc

SEQ ID NO: 38 - DNA, 18 bp, synthetic construct
  misc_feature 1..18: note = Single strand DNA oligonucleotide
  source 1..18: mol_type = other DNA
tcacctccctccacacat

SEQ ID NO: 39 - DNA, 20 bp, synthetic construct
  misc_feature 1..20: note = gRNA sequence
  source 1..20: mol_type = other DNA
cactccaataatgccggtac

SEQ ID NO: 40 - DNA, 21 bp, synthetic construct
  misc_feature 1..21: note = Single strand DNA oligonucleotide
  source 1..21: mol_type = other DNA
atctcttcttgcacagtggac

SEQ ID NO: 41 - DNA, 20 bp, synthetic construct
  misc_feature 1..20: note = Single strand DNA oligonucleotide
  source 1..20: mol_type = other DNA
acggtgttctgtttctcctg

SEQ ID NO: 42 - DNA, 20 bp, synthetic construct
  misc_feature 1..20: note = gRNA sequence
  source 1..20: mol_type = other DNA
agaggtgcacggtcccattg

SEQ ID NO: 43 - DNA, 21 bp, synthetic construct
  misc_feature 1..21: note = Single strand DNA oligonucleotide
  source 1..21: mol_type = other DNA
gaagaaccagtaccggcatta

SEQ ID NO: 44 - DNA, 21 bp, synthetic construct
  misc_feature 1..21: note = Single strand DNA oligonucleotide
  source 1..21: mol_type = other DNA
gttgtcagacccacagaatac

SEQ ID NO: 45 - DNA, 20 bp, synthetic construct
  misc_feature 1..20: note = gRNA sequence
  source 1..20: mol_type = other DNA
ttggactggtccctcaccta

SEQ ID NO: 46 - DNA, 22 bp, synthetic construct
  misc_feature 1..22: note = Single strand DNA oligonucleotide
  source 1..22: mol_type = other DNA
tctcttgatggtgtctcctcta

SEQ ID NO: 47 - DNA, 22 bp, synthetic construct
  misc_feature 1..22: note = Single strand DNA oligonucleotide
  source 1..22: mol_type = other DNA
actggaagaagcagagaaagaa